European Patent Application EP 4 538 370 A1, published April 16, 2025. Title: Truncated forms of IgA protease, fusion proteins comprising the same, and uses thereof. Applicant: Peking University First Hospital. The sequence listing filed with the application follows.

SEQUENCE LISTING (31 sequences)

SEQ ID NO: 1 - protein, 2004 aa, Streptococcus pneumoniae
MEKYFGEKQERFSFRKLSVGLVSATISSLFFMSVLASSSVDAQETAGVHYKYVADSELSSEEKKQLVYDIPTYVENDDETYYLVYKLNSQNQLAELPNTGSKNERQALVAGASLAAMGILIFAVSKKKVKNKTVLHLVLVAGIGNGVLVSVHALENHLLLNYNTDYELTSGEKLPLPKEISGYTYIGYIKEGKTTSESEVSNQKSSVATPTKQQKVDYNVTPNFVDHPSTVQAIQEQTPVSSTKPTEVQVVEKPFSTELINPRKEEKQSSDSQEQLAEHKNLETKKEEKISPKEKTGVNTLNPQDEVLSGQLNKPELLYREETMETKIDFQEEIQENPDLAEGTVRVKQEGKLGKKVEIVRIFSVNKEEVSREIVSTSTTAPSPRIVEKGTKKTQVIKEQPETGVEHKDVQSGAIVEPAIQPELPEAVVSDKGEPEVQPTLPEAVVTDKGETEVQPESPDTVVSDKGEPEQVAPLPEYKGNIEQVKPETPVEKTKEQGPEKTEEVPVKPTEETPVNPNEGTTEGTSIQEAENPVQPAEESTTNSEKVSPDTSSKNTGEVSSNPSDSTTSVGESNKPEHNDSKNENSEKTVEEVPVNPNEGTVEGTSNQETEKPVQPAEETQTNSGKIANENTGEVSNKPSDSKPPVEESNQPEKNGTATKPENSGNTTSENGQTEPEPSNGNSTEDVSTESNTSNSNGNEEIKQENELDPDKKVEEPEKTLELRNVSDLELYSLSNGTYKQHISLEQVPSNPNSYFVKVKSSSFKDVYLPVASISEERKNDKILYKITAKVEKLQQEIESRYKDNFTFYLAKKGTEETTNFTSFSNLVKAINQNPSGTYHLAASLNANEVELGPDERSYIKDTFTGRLIGEKDGKNYAIYNLKKPLFENLSGATVEKLSLKNVAISGKDDIGSLANEAQNNTKIKQVHVDGVLAGERGIGGLLAKAEQSSITESSFKGRIINTYETTAAYNIGGMVGHLTGDKALLTKSKATVAISSNTNTSDQTVGGLAGLVDRDAQIQDSYAEGDINNVKHFGRVAGVAGNLWDRTSGDVRHAGSLTNVLSDVNVTNGNAITGYHYNEMKVKDTFSSKANRVYNVTLVKDEVVSKESFEERGTMLDASQIASKKAEINPLILPTVEPLSTSGKKDSDFSKVAYYQAKRNLTYKNIEKLLPFYNKATIVKYGNLVNENSLLYQKELLSAVMMKDNQVITDIVSNKQTANKLLLHYKDDLSEKLDLKYQNDFAKLAEYSLGNTGLLYTPNQFLYDQTSIIKQVLPDLQKVDYHSEAIRKTLGISPNVKQTELYLEDQFAKTKQQLEDSLKKLLSADAGLASANPVTEGYLVDKIKRNKEALLLGLTYLERWYNFSYGQVNVKDLVLYHLDFFGKGNASPLDTLIELGKSGFNNLLAKNNVDTYGISLASQHGTTDLFSTLEHYRKVFLPNTSNNDWFKSETKAYIVEEKSTIEEVKTKQGLAGTKYSIGVYDRITSATWKYRNMVLPLLTLPERSVFVISTMSSLGFGAYDRYRSSDHKAGKALNDFVEENARETAKRQRDHYDYWYRILDDNAREKLYRNILLYDAYKFGDDNTVGKATEVADFDNPNPAMQHFFGPVGNKVGHNQHGAYATGDAVYYMGYRMLDKDGAITYTHEMTHDSDQDIYLGGYGRRSGLGPEFFAKGLLQAPDHPDDATITINSILKHSKSDSTESRRLQVLDPTTRFNNADDLKQYVHNMFDVVYMLEYLEGNSILKLDTNQKQQLLRKVTNEYHPDPDGNKVYATNVVRNLTVEEVERLRSFNDLIDNNILSSREYASGKYERNGYFTIKLFAPIYAALSNDIGTPGDLMGRRIAYELLAAKGFKDGMVPYISNQYEEEAKQKGKTINLYGKTRGLVTDDLVLEKVFNNQYHTWSEFKKAMYQERQDQFDRLNKVTFNDTTQPWQTFAKKTTSSVDELQKLMDVAVRKDAEHNYYHWNNYNPDIDSEVHKLKRAIFKAYLDQTNDFRSSIFENKK

SEQ ID NO: 2 - protein, 1340 aa, synthetic construct
GNTTSENGQTEPEPSNGNSTEDVSTESNTSNSNGNEEIKQENELDPDKKVEEPEKTLELRNVSDLELYSLSNGTYKQHISLEQVPSNPNSYFVKVKSSSFKDVYLPVASISEERKNDKILYKITAKVEKLQQEIESRYKDNFTFYLAKKGTEETTNFTSFSNLVKAINQNPSGTYHLAASLNANEVELGPDERSYIKDTFTGRLIGEKDGKNYAIYNLKKPLFENLSGATVEKLSLKNVAISGKDDIGSLANEAQNNTKIKQVHVDGVLAGERGIGGLLAKAEQSSITESSFKGRIINTYETTAAYNIGGMVGHLTGDKALLTKSKATVAISSNTNTSDQTVGGLAGLVDRDAQIQDSYAEGDINNVKHFGRVAGVAGNLWDRTSGDVRHAGSLTNVLSDVNVTNGNAITGYHYNEMKVKDTFSSKANRVYNVTLVKDEVVSKESFEERGTMLDASQIASKKAEINPLILPTVEPLSTSGKKDSDFSKVAYYQAKRNLTYKNIEKLLPFYNKATIVKYGNLVNENSLLYQKELLSAVMMKDNQVITDIVSNKQTANKLLLHYKDDLSEKLDLKYQNDFAKLAEYSLGNTGLLYTPNQFLYDQTSIIKQVLPDLQKVDYHSEAIRKTLGISPNVKQTELYLEDQFAKTKQQLEDSLKKLLSADAGLASANPVTEGYLVDKIKRNKEALLLGLTYLERWYNFSYGQVNVKDLVLYHLDFFGKGNASPLDTLIELGKSGFNNLLAKNNVDTYGISLASQHGTTDLFSTLEHYRKVFLPNTSNNDWFKSETKAYIVEEKSTIEEVKTKQGLAGTKYSIGVYDRITSATWKYRNMVLPLLTLPERSVFVISTMSSLGFGAYDRYRSSDHKAGKALNDFVEENARETAKRQRDHYDYWYRILDDNAREKLYRNILLYDAYKFGDDNTVGKATEVADFDNPNPAMQHFFGPVGNKVGHNQHGAYATGDAVYYMGYRMLDKDGAITYTHEMTHDSDQDIYLGGYGRRSGLGPEFFAKGLLQAPDHPDDATITINSILKHSKSDSTESRRLQVLDPTTRFNNADDLKQYVHNMFDVVYMLEYLEGNSILKLDTNQKQQLLRKVTNEYHPDPDGNKVYATNVVRNLTVEEVERLRSFNDLIDNNILSSREYASGKYERNGYFTIKLFAPIYAALSNDIGTPGDLMGRRIAYELLAAKGFKDGMVPYISNQYEEEAKQKGKTINLYGKTRGLVTDDLVLEKVFNNQYHTWSEFKKAMYQERQDQFDRLNKVTFNDTTQPWQTFAKKTTSSVDELQKLMDVAVRKDAEHNYYHWNNYNPDIDSEVHKLKRAIFKAYLDQTNDFRSSIFENKK

SEQ ID NO: 3 - protein, 1260 aa, synthetic construct
LEQVPSNPNSYFVKVKSSSFKDVYLPVASISEERKNDKILYKITAKVEKLQQEIESRYKDNFTFYLAKKGTEETTNFTSFSNLVKAINQNPSGTYHLAASLNANEVELGPDERSYIKDTFTGRLIGEKDGKNYAIYNLKKPLFENLSGATVEKLSLKNVAISGKDDIGSLANEAQNNTKIKQVHVDGVLAGERGIGGLLAKAEQSSITESSFKGRIINTYETTAAYNIGGMVGHLTGDKALLTKSKATVAISSNTNTSDQTVGGLAGLVDRDAQIQDSYAEGDINNVKHFGRVAGVAGNLWDRTSGDVRHAGSLTNVLSDVNVTNGNAITGYHYNEMKVKDTFSSKANRVYNVTLVKDEVVSKESFEERGTMLDASQIASKKAEINPLILPTVEPLSTSGKKDSDFSKVAYYQAKRNLTYKNIEKLLPFYNKATIVKYGNLVNENSLLYQKELLSAVMMKDNQVITDIVSNKQTANKLLLHYKDDLSEKLDLKYQNDFAKLAEYSLGNTGLLYTPNQFLYDQTSIIKQVLPDLQKVDYHSEAIRKTLGISPNVKQTELYLEDQFAKTKQQLEDSLKKLLSADAGLASANPVTEGYLVDKIKRNKEALLLGLTYLERWYNFSYGQVNVKDLVLYHLDFFGKGNASPLDTLIELGKSGFNNLLAKNNVDTYGISLASQHGTTDLFSTLEHYRKVFLPNTSNNDWFKSETKAYIVEEKSTIEEVKTKQGLAGTKYSIGVYDRITSATWKYRNMVLPLLTLPERSVFVISTMSSLGFGAYDRYRSSDHKAGKALNDFVEENARETAKRQRDHYDYWYRILDDNAREKLYRNILLYDAYKFGDDNTVGKATEVADFDNPNPAMQHFFGPVGNKVGHNQHGAYATGDAVYYMGYRMLDKDGAITYTHEMTHDSDQDIYLGGYGRRSGLGPEFFAKGLLQAPDHPDDATITINSILKHSKSDSTESRRLQVLDPTTRFNNADDLKQYVHNMFDVVYMLEYLEGNSILKLDTNQKQQLLRKVTNEYHPDPDGNKVYATNVVRNLTVEEVERLRSFNDLIDNNILSSREYASGKYERNGYFTIKLFAPIYAALSNDIGTPGDLMGRRIAYELLAAKGFKDGMVPYISNQYEEEAKQKGKTINLYGKTRGLVTDDLVLEKVFNNQYHTWSEFKKAMYQERQDQFDRLNKVTFNDTTQPWQTFAKKTTSSVDELQKLMDVAVRKDAEHNYYHWNNYNPDIDSEVHKLKRAIFKAYLDQTNDFRSSIFENKK

SEQ ID NO: 4 - protein, 1160 aa, synthetic construct
LNANEVELGPDERSYIKDTFTGRLIGEKDGKNYAIYNLKKPLFENLSGATVEKLSLKNVAISGKDDIGSLANEAQNNTKIKQVHVDGVLAGERGIGGLLAKAEQSSITESSFKGRIINTYETTAAYNIGGMVGHLTGDKALLTKSKATVAISSNTNTSDQTVGGLAGLVDRDAQIQDSYAEGDINNVKHFGRVAGVAGNLWDRTSGDVRHAGSLTNVLSDVNVTNGNAITGYHYNEMKVKDTFSSKANRVYNVTLVKDEVVSKESFEERGTMLDASQIASKKAEINPLILPTVEPLSTSGKKDSDFSKVAYYQAKRNLTYKNIEKLLPFYNKATIVKYGNLVNENSLLYQKELLSAVMMKDNQVITDIVSNKQTANKLLLHYKDDLSEKLDLKYQNDFAKLAEYSLGNTGLLYTPNQFLYDQTSIIKQVLPDLQKVDYHSEAIRKTLGISPNVKQTELYLEDQFAKTKQQLEDSLKKLLSADAGLASANPVTEGYLVDKIKRNKEALLLGLTYLERWYNFSYGQVNVKDLVLYHLDFFGKGNASPLDTLIELGKSGFNNLLAKNNVDTYGISLASQHGTTDLFSTLEHYRKVFLPNTSNNDWFKSETKAYIVEEKSTIEEVKTKQGLAGTKYSIGVYDRITSATWKYRNMVLPLLTLPERSVFVISTMSSLGFGAYDRYRSSDHKAGKALNDFVEENARETAKRQRDHYDYWYRILDDNAREKLYRNILLYDAYKFGDDNTVGKATEVADFDNPNPAMQHFFGPVGNKVGHNQHGAYATGDAVYYMGYRMLDKDGAITYTHEMTHDSDQDIYLGGYGRRSGLGPEFFAKGLLQAPDHPDDATITINSILKHSKSDSTESRRLQVLDPTTRFNNADDLKQYVHNMFDVVYMLEYLEGNSILKLDTNQKQQLLRKVTNEYHPDPDGNKVYATNVVRNLTVEEVERLRSFNDLIDNNILSSREYASGKYERNGYFTIKLFAPIYAALSNDIGTPGDLMGRRIAYELLAAKGFKDGMVPYISNQYEEEAKQKGKTINLYGKTRGLVTDDLVLEKVFNNQYHTWSEFKKAMYQERQDQFDRLNKVTFNDTTQPWQTFAKKTTSSVDELQKLMDVAVRKDAEHNYYHWNNYNPDIDSEVHKLKRAIFKAYLDQTNDFRSSIFENKK

SEQ ID NO: 5 - protein, 2193 aa, synthetic construct
TCPPCPAPELLGGPSVFLFPPKPKDTLMISRTPEVTCVVVDVSHEDPEVKFNWYVDGVEVHNAKTKPREEQYNSTYRVVSVLTVLHQDWLNGKEYKCKVSNKALPAPIEKTISKAKGQPREPQVYTLPPSRDELTKNQVSLTCLVKGFYPSDIAVEWESNGQPENNYKTTPPVLDSDGSFFLYSKLTVDKSRWQQGNVFSCSVMHEALHNHYTQKSLSLSPGKGGGGGGSRQETAGVHYKYVADSELSSEEKKQLVYDIPTYVENDDETYYLVYKLNSQNQLAELPNTGSKNERQALVAGASLAAMGILIFAVSKKKVKNKTVLHLVLVAGIGNGVLVSVHALENHLLLNYNTDYELTSGEKLPLPKEISGYTYIGYIKEGKTTSESEVSNQKSSVATPTKQQKVDYNVTPNFVDHPSTVQAIQEQTPVSSTKPTEVQVVEKPFSTELINPRKEEKQSSDSQEQLAEHKNLETKKEEKISPKEKTGVNTLNPQDEVLSGQLNKPELLYREETMETKIDFQEEIQENPDLAEGTVRVKQEGKLGKKVEIVRIFSVNKEEVSREIVSTSTTAPSPRIVEKGTKKTQVIKEQPETGVEHKDVQSGAIVEPAIQPELPEAVVSDKGEPEVQPTLPEAVVTDKGETEVQPESPDTVVSDKGEPEQVAPLPEYKGNIEQVKPETPVEKTKEQGPEKTEEVPVKPTEETPVNPNEGTTEGTSIQEAENPVQPAEESTTNSEKVSPDTSSKNTGEVSSNPSDSTTSVGESNKPEHNDSKNENSEKTVEEVPVNPNEGTVEGTSNQETEKPVQPAEETQTNSGKIANENTGEVSNKPSDSKPPVEESNQPEKNGTATKPENSGNTTSENGQTEPEPSNGNSTEDVSTESNTSNSNGNEEIKQENELDPDKKVEEPEKTLELRNVSDLELYSLSNGTYKQHISLEQVPSNPNSYFVKVKSSSFKDVYLPVASISEERKNDKILYKITAKVEKLQQEIESRYKDNFTFYLAKKGTEETTNFTSFSNLVKAINQNPSGTYHLAASLNANEVELGPDERSYIKDTFTGRLIGEKDGKNYAIYNLKKPLFENLSGATVEKLSLKNVAISGKDDIGSLANEAQNNTKIKQVHVDGVLAGERGIGGLLAKAEQSSITESSFKGRIINTYETTAAYNIGGMVGHLTGDKALLTKSKATVAISSNTNTSDQTVGGLAGLVDRDAQIQDSYAEGDINNVKHFGRVAGVAGNLWDRTSGDVRHAGSLTNVLSDVNVTNGNAITGYHYNEMKVKDTFSSKANRVYNVTLVKDEVVSKESFEERGTMLDASQIASKKAEINPLILPTVEPLSTSGKKDSDFSKVAYYQAKRNLTYKNIEKLLPFYNKATIVKYGNLVNENSLLYQKELLSAVMMKDNQVITDIVSNKQTANKLLLHYKDDLSEKLDLKYQNDFAKLAEYSLGNTGLLYTPNQFLYDQTSIIKQVLPDLQKVDYHSEAIRKTLGISPNVKQTELYLEDQFAKTKQQLEDSLKKLLSADAGLASANPVTEGYLVDKIKRNKEALLLGLTYLERWYNFSYGQVNVKDLVLYHLDFFGKGNASPLDTLIELGKSGFNNLLAKNNVDTYGISLASQHGTTDLFSTLEHYRKVFLPNTSNNDWFKSETKAYIVEEKSTIEEVKTKQGLAGTKYSIGVYDRITSATWKYRNMVLPLLTLPERSVFVISTMSSLGFGAYDRYRSSDHKAGKALNDFVEENARETAKRQRDHYDYWYRILDDNAREKLYRNILLYDAYKFGDDNTVGKATEVADFDNPNPAMQHFFGPVGNKVGHNQHGAYATGDAVYYMGYRMLDKDGAITYTHEMTHDSDQDIYLGGYGRRSGLGPEFFAKGLLQAPDHPDDATITINSILKHSKSDSTESRRLQVLDPTTRFNNADDLKQYVHNMFDVVYMLEYLEGNSILKLDTNQKQQLLRKVTNEYHPDPDGNKVYATNVVRNLTVEEVERLRSFNDLIDNNILSSREYASGKYERNGYFTIKLFAPIYAALSNDIGTPGDLMGRRIAYELLAAKGFKDGMVPYISNQYEEEAKQKGKTINLYGKTRGLVTDDLVLEKVFNNQYHTWSEFKKAMYQERQDQFDRLNKVTFNDTTQPWQTFAKKTTSSVDELQKLMDVAVRKDAEHNYYHWNNYNPDIDSEVHKLKRAIFKAYLDQTNDFRSSIFENKK

SEQ ID NO: 6 - protein, 1571 aa, synthetic construct
TCPPCPAPELLGGPSVFLFPPKPKDTLMISRTPEVTCVVVDVSHEDPEVKFNWYVDGVEVHNAKTKPREEQYNSTYRVVSVLTVLHQDWLNGKEYKCKVSNKALPAPIEKTISKAKGQPREPQVYTLPPSRDELTKNQVSLTCLVKGFYPSDIAVEWESNGQPENNYKTTPPVLDSDGSFFLYSKLTVDKSRWQQGNVFSCSVMHEALHNHYTQKSLSLSPGKGGGGGGSRGNTTSENGQTEPEPSNGNSTEDVSTESNTSNSNGNEEIKQENELDPDKKVEEPEKTLELRNVSDLELYSLSNGTYKQHISLEQVPSNPNSYFVKVKSSSFKDVYLPVASISEERKNDKILYKITAKVEKLQQEIESRYKDNFTFYLAKKGTEETTNFTSFSNLVKAINQNPSGTYHLAASLNANEVELGPDERSYIKDTFTGRLIGEKDGKNYAIYNLKKPLFENLSGATVEKLSLKNVAISGKDDIGSLANEAQNNTKIKQVHVDGVLAGERGIGGLLAKAEQSSITESSFKGRIINTYETTAAYNIGGMVGHLTGDKALLTKSKATVAISSNTNTSDQTVGGLAGLVDRDAQIQDSYAEGDINNVKHFGRVAGVAGNLWDRTSGDVRHAGSLTNVLSDVNVTNGNAITGYHYNEMKVKDTFSSKANRVYNVTLVKDEVVSKESFEERGTMLDASQIASKKAEINPLILPTVEPLSTSGKKDSDFSKVAYYQAKRNLTYKNIEKLLPFYNKATIVKYGNLVNENSLLYQKELLSAVMMKDNQVITDIVSNKQTANKLLLHYKDDLSEKLDLKYQNDFAKLAEYSLGNTGLLYTPNQFLYDQTSIIKQVLPDLQKVDYHSEAIRKTLGISPNVKQTELYLEDQFAKTKQQLEDSLKKLLSADAGLASANPVTEGYLVDKIKRNKEALLLGLTYLERWYNFSYGQVNVKDLVLYHLDFFGKGNASPLDTLIELGKSGFNNLLAKNNVDTYGISLASQHGTTDLFSTLEHYRKVFLPNTSNNDWFKSETKAYIVEEKSTIEEVKTKQGLAGTKYSIGVYDRITSATWKYRNMVLPLLTLPERSVFVISTMSSLGFGAYDRYRSSDHKAGKALNDFVEENARETAKRQRDHYDYWYRILDDNAREKLYRNILLYDAYKFGDDNTVGKATEVADFDNPNPAMQHFFGPVGNKVGHNQHGAYATGDAVYYMGYRMLDKDGAITYTHEMTHDSDQDIYLGGYGRRSGLGPEFFAKGLLQAPDHPDDATITINSILKHSKSDSTESRRLQVLDPTTRFNNADDLKQYVHNMFDVVYMLEYLEGNSILKLDTNQKQQLLRKVTNEYHPDPDGNKVYATNVVRNLTVEEVERLRSFNDLIDNNILSSREYASGKYERNGYFTIKLFAPIYAALSNDIGTPGDLMGRRIAYELLAAKGFKDGMVPYISNQYEEEAKQKGKTINLYGKTRGLVTDDLVLEKVFNNQYHTWSEFKKAMYQERQDQFDRLNKVTFNDTTQPWQTFAKKTTSSVDELQKLMDVAVRKDAEHNYYHWNNYNPDIDSEVHKLKRAIFKAYLDQTNDFRSSIFENKK

SEQ ID NO: 7 - protein, 1580 aa, synthetic construct
GNTTSENGQTEPEPSNGNSTEDVSTESNTSNSNGNEEIKQENELDPDKKVEEPEKTLELRNVSDLELYSLSNGTYKQHISLEQVPSNPNSYFVKVKSSSFKDVYLPVASISEERKNDKILYKITAKVEKLQQEIESRYKDNFTFYLAKKGTEETTNFTSFSNLVKAINQNPSGTYHLAASLNANEVELGPDERSYIKDTFTGRLIGEKDGKNYAIYNLKKPLFENLSGATVEKLSLKNVAISGKDDIGSLANEAQNNTKIKQVHVDGVLAGERGIGGLLAKAEQSSITESSFKGRIINTYETTAAYNIGGMVGHLTGDKALLTKSKATVAISSNTNTSDQTVGGLAGLVDRDAQIQDSYAEGDINNVKHFGRVAGVAGNLWDRTSGDVRHAGSLTNVLSDVNVTNGNAITGYHYNEMKVKDTFSSKANRVYNVTLVKDEVVSKESFEERGTMLDASQIASKKAEINPLILPTVEPLSTSGKKDSDFSKVAYYQAKRNLTYKNIEKLLPFYNKATIVKYGNLVNENSLLYQKELLSAVMMKDNQVITDIVSNKQTANKLLLHYKDDLSEKLDLKYQNDFAKLAEYSLGNTGLLYTPNQFLYDQTSIIKQVLPDLQKVDYHSEAIRKTLGISPNVKQTELYLEDQFAKTKQQLEDSLKKLLSADAGLASANPVTEGYLVDKIKRNKEALLLGLTYLERWYNFSYGQVNVKDLVLYHLDFFGKGNASPLDTLIELGKSGFNNLLAKNNVDTYGISLASQHGTTDLFSTLEHYRKVFLPNTSNNDWFKSETKAYIVEEKSTIEEVKTKQGLAGTKYSIGVYDRITSATWKYRNMVLPLLTLPERSVFVISTMSSLGFGAYDRYRSSDHKAGKALNDFVEENARETAKRQRDHYDYWYRILDDNAREKLYRNILLYDAYKFGDDNTVGKATEVADFDNPNPAMQHFFGPVGNKVGHNQHGAYATGDAVYYMGYRMLDKDGAITYTHEMTHDSDQDIYLGGYGRRSGLGPEFFAKGLLQAPDHPDDATITINSILKHSKSDSTESRRLQVLDPTTRFNNADDLKQYVHNMFDVVYMLEYLEGNSILKLDTNQKQQLLRKVTNEYHPDPDGNKVYATNVVRNLTVEEVERLRSFNDLIDNNILSSREYASGKYERNGYFTIKLFAPIYAALSNDIGTPGDLMGRRIAYELLAAKGFKDGMVPYISNQYEEEAKQKGKTINLYGKTRGLVTDDLVLEKVFNNQYHTWSEFKKAMYQERQDQFDRLNKVTFNDTTQPWQTFAKKTTSSVDELQKLMDVAVRKDAEHNYYHWNNYNPDIDSEVHKLKRAIFKAYLDQTNDFRSSIFENKKRSGGGGSHHHHHHHHHHTCPPCPAPELLGGPSVFLFPPKPKDTLMISRTPEVTCVVVDVSHEDPEVKFNWYVDGVEVHNAKTKPREEQYNSTYRVVSVLTVLHQDWLNGKEYKCKVSNKALPAPIEKTISKAKGQPREPQVYTLPPSRDELTKNQVSLTCLVKGFYPSDIAVEWESNGQPENNYKTTPPVLDSDGSFFLYSKLTVDKSRWQQGNVFSCSVMHEALHNHYTQKSLSLSPGK

SEQ ID NO: 8 - protein, 1576 aa, synthetic construct
GNTTSENGQTEPEPSNGNSTEDVSTESNTSNSNGNEEIKQENELDPDKKVEEPEKTLELRNVSDLELYSLSNGTYKQHISLEQVPSNPNSYFVKVKSSSFKDVYLPVASISEERKNDKILYKITAKVEKLQQEIESRYKDNFTFYLAKKGTEETTNFTSFSNLVKAINQNPSGTYHLAASLNANEVELGPDERSYIKDTFTGRLIGEKDGKNYAIYNLKKPLFENLSGATVEKLSLKNVAISGKDDIGSLANEAQNNTKIKQVHVDGVLAGERGIGGLLAKAEQSSITESSFKGRIINTYETTAAYNIGGMVGHLTGDKALLTKSKATVAISSNTNTSDQTVGGLAGLVDRDAQIQDSYAEGDINNVKHFGRVAGVAGNLWDRTSGDVRHAGSLTNVLSDVNVTNGNAITGYHYNEMKVKDTFSSKANRVYNVTLVKDEVVSKESFEERGTMLDASQIASKKAEINPLILPTVEPLSTSGKKDSDFSKVAYYQAKRNLTYKNIEKLLPFYNKATIVKYGNLVNENSLLYQKELLSAVMMKDNQVITDIVSNKQTANKLLLHYKDDLSEKLDLKYQNDFAKLAEYSLGNTGLLYTPNQFLYDQTSIIKQVLPDLQKVDYHSEAIRKTLGISPNVKQTELYLEDQFAKTKQQLEDSLKKLLSADAGLASANPVTEGYLVDKIKRNKEALLLGLTYLERWYNFSYGQVNVKDLVLYHLDFFGKGNASPLDTLIELGKSGFNNLLAKNNVDTYGISLASQHGTTDLFSTLEHYRKVFLPNTSNNDWFKSETKAYIVEEKSTIEEVKTKQGLAGTKYSIGVYDRITSATWKYRNMVLPLLTLPERSVFVISTMSSLGFGAYDRYRSSDHKAGKALNDFVEENARETAKRQRDHYDYWYRILDDNAREKLYRNILLYDAYKFGDDNTVGKATEVADFDNPNPAMQHFFGPVGNKVGHNQHGAYATGDAVYYMGYRMLDKDGAITYTHEMTHDSDQDIYLGGYGRRSGLGPEFFAKGLLQAPDHPDDATITINSILKHSKSDSTESRRLQVLDPTTRFNNADDLKQYVHNMFDVVYMLEYLEGNSILKLDTNQKQQLLRKVTNEYHPDPDGNKVYATNVVRNLTVEEVERLRSFNDLIDNNILSSREYASGKYERNGYFTIKLFAPIYAALSNDIGTPGDLMGRRIAYELLAAKGFKDGMVPYISNQYEEEAKQKGKTINLYGKTRGLVTDDLVLEKVFNNQYHTWSEFKKAMYQERQDQFDRLNKVTFNDTTQPWQTFAKKTTSSVDELQKLMDVAVRKDAEHNYYHWNNYNPDIDSEVHKLKRAIFKAYLDQTNDFRSSIFENKKRSGGGGSESKYGPPCPSCPAPEFLGGPSVFLFPPKPKDTLMISRTPEVTCVVVDVSQEDPEVQFNWYVDGVEVHNAKTKPREEQFNSTYRVVSVLTVLHQDWLNGKEYKCKVSNKGLPSSIEKTISKAKGQPREPQVYTLPPSQEEMTKNQVSLTCLVKGFYPSDIAVEWESNGQPENNYKTTPPVLDSDGSFFLYSRLTVDKSRWQEGNVFSCSVMHEALHNHYTQKSLSLSLGK

SEQ ID NO: 9 - DNA, 6579 bp, synthetic construct
  source 1..6579: mol_type = other DNA
acatgcccaccgtgcccagcacctgaactcctggggggaccgtcagtcttcctcttccccccaaaacccaaggacaccctcatgatctcccggacccctgaggtcacatgcgtggtggtggacgtgagccacgaagaccctgaggtcaagttcaactggtacgtggacggcgtggaggtgcataatgccaagacaaagccgcgggaggagcagtacaacagcacgtaccgggtggtcagcgtcctcaccgtcctgcaccaggactggctgaatggcaaggagtacaagtgcaaggtctccaacaaagccctcccagcccccatcgagaaaaccatctccaaagccaaagggcagccccgagaaccacaggtgtacaccctgcccccatcccgggatgagctgaccaagaaccaggtcagcctgacctgcctggtcaaaggcttctatcccagcgacatcgccgtggagtgggagagcaatgggcagccggagaacaactacaagaccacgcctcccgtgctggactccgacggctccttcttcctctacagcaagctcaccgtggacaagagcaggtggcagcaggggaacgtcttctcatgctccgtgatgcatgaggctctgcacaaccactacacgcagaagagcctctccctgtctccgggtaaaggtggcggtggcggcggttctagacaagaaacggcaggtgtgcattacaaatacgtggcagatagcgaactgagcagcgaagaaaaaaaacaactggtctacgacatcccgacctacgtcgaaaatgatgacgaaacgtattacctggtgtataaactgaattcacagaaccaactggcagaactgccgaataccggctcgaaaaacgaacgtcaggctctggtggcaggtgctagcctggcagcaatgggtattctgatctttgccgtgagcaagaaaaaagttaaaaacaaaaccgtcctgcatctggtcctggtggcaggcattggtaatggcgttctggtcagcgtgcatgctctggaaaaccacctgctgctgaactacaataccgattatgaactgacgagcggtgaaaaactgccgctgccgaaagaaatctctggctatacctacattggttacatcaaagaaggcaaaaccacgtcggaaagcgaagtctccaaccagaaaagctctgtggcaaccccgacgaaacagcaaaaagttgactataatgtcaccccgaacttcgttgatcatccgtctaccgtccaagcgattcaggaacaaacgccggtcagctccaccaaaccgacggaagtgcaggtggttgaaaaaccgttttcaaccgaactgatcaatccgcgtaaagaagaaaaacagtcatcggattcgcaggaacaactggcggaacacaaaaacctggaaaccaaaaaagaagaaaaaatcagcccgaaagaaaaaaccggcgtgaatacgctgaacccgcaggatgaagttctgtctggtcaactgaataaaccggaactgctgtatcgtgaagaaaccatggaaacgaaaattgacttccaggaagaaatccaagaaaacccggatctggcggaaggcaccgttcgcgtcaaacaggaaggtaaactgggcaaaaaagttgaaattgtccgtatcttttccgtgaataaagaagaagtttcacgcgaaattgtctctaccagtaccacggcaccgagcccgcgtattgtcgaaaaaggtaccaagaaaacccaggtgatcaaagaacaacctgaaaccggcgtggaacataaagatgttcagagtggtgctattgtggaaccggcgatccaaccggaactgccggaagcggtcgtgtccgataaaggcgaaccggaagttcagccgaccctgccggaagccgttgtcaccgacaaaggtgaaacggaagtgcagccggaatccccggacaccgtggtttcagataaaggtgaaccggaacaggttgcaccgctgccggaatacaagggtaacatcgaacaagtgaaaccggaaaccccggtggaaaaaacgaaagaacagggcccggaaaaaaccgaagaagtgccggttaaaccgaccgaagaaacgccggtgaacccgaatgaaggtaccacggaaggcaccagcatccaggaagccgaaaatccggttcaaccggcagaagaatcaaccacgaactcggaaaaagtcagcccggacaccagctctaaaaatacgggcgaagttagttccaacccgtccgattcaaccacgtctgtcggtgaaagtaataaaccggaacacaacgactccaaaaacgaaaattcagaaaaaaccgtcgaagaagtcccggttaatccgaatgaaggtaccgtggaaggcacgagcaatcaggaaaccgaaaaaccggttcagccggcagaagaaacccaaacgaatagtggcaaaattgctaacgaaaataccggtgaagtgtccaacaaaccgtcggatagcaaaccgccggttgaagaaagcaatcagccggagaaaaacggcaccgcgacgaaaccggaaaattcgggcaacaccacgagcgaaaacggtcagaccgaaccggaaccgtccaacggcaattcaacggaagatgttagtaccgaatccaatacgtctaacagtaacggtaacgaagaaatcaaacaggaaaacgaactggatccggacaaaaaagtcgaagaaccggaaaaaaccctggaactgcgcaatgtgagcgatctggaactgtattccctgtcaaacggcacgtacaaacagcatatctctctggaacaagttccgtcgaatccgaacagctactttgttaaagtcaaatcatcgagcttcaaagatgtgtatctgccggttgcatcgatcagcgaagaacgtaaaaatgacaaaatcctgtacaaaatcaccgctaaagtggaaaaactgcagcaagaaatcgaaagccgctataaagataactttacgttctacctggcgaaaaaaggtaccgaagaaaccacgaattttacgtctttcagtaacctggttaaagcgattaatcagaacccgtcaggcacctaccacctggcagcttcgctgaatgccaacgaagtggaactgggtccggacgaacgtagctatattaaagataccttcacgggtcgcctgatcggcgaaaaagatggtaaaaactacgccatctacaacctgaaaaaaccgctgtttgaaaatctgtctggcgcgaccgttgaaaaactgtcgctgaaaaacgtcgccattagcggtaaagatgacatcggctctctggcgaatgaagcccagaacaataccaaaatcaaacaagtgcatgttgatggcgtgctggcaggtgaacgtggcattggcggtctgctggcgaaagccgaacagtctagtatcaccgaatcctcatttaaaggtcgcattatcaatacgtatgaaaccacggcggcctacaacattggcggtatggttggccacctgaccggtgataaagccctgctgaccaaaagcaaagcaacggtggctatctcgagcaataccaacacgtctgatcagaccgttggcggtctggctggtctggtcgatcgtgacgcgcagattcaagactcttatgccgaaggcgatatcaacaatgttaaacattttggtcgcgtggcgggtgttgccggcaatctgtgggaccgtaccagtggcgatgttcgccacgcaggttcgctgacgaatgtcctgagcgatgtcaacgtgaccaatggtaacgctattacgggctaccattacaacgaaatgaaagtgaaagataccttctctagtaaagcgaatcgtgtctataacgtgacgctggttaaagatgaagtcgtgtcaaaagaatcgtttgaagaacgcggcaccatgctggacgcatctcagatcgctagtaaaaaagcggaaattaacccgctgatcctgccgaccgttgaaccgctgtccacgtcaggtaaaaaagatagcgacttctctaaagtggcctattaccaggcaaaacgtaacctgacctacaaaaacatcgaaaaactgctgccgttctacaacaaagccacgatcgtcaaatacggcaacctggtgaatgaaaacagcctgctgtatcagaaagaactgctgtctgcggtgatgatgaaagacaatcaggtcattaccgatatcgtgagtaataaacaaacggccaacaaactgctgctgcattataaagatgacctgtccgaaaaactggacctgaaatatcagaacgatttcgcaaaactggctgaatactcactgggtaataccggcctgctgtatacgccgaaccagtttctgtacgatcaaacctcgattatcaaacaggtgctgccggacctgcaaaaagttgattaccactcagaagcaattcgcaaaaccctgggtatctcgccgaatgtgaaacagacggaactgtatctggaagatcaatttgctaaaaccaaacagcaactggaagactctctgaaaaaactgctgagtgcagatgctggcctggcgtctgccaatccggttaccgaaggttacctggtcgataaaattaaacgtaacaaagaagccctgctgctgggcctgacctatctggaacgctggtacaatttcagctatggtcaggttaacgtcaaagacctggtgctgtatcatctggatttctttggtaaaggcaacgcaagtccgctggataccctgattgaactgggtaaatccggctttaacaatctgctggcgaaaaacaatgttgacacctacggcatcagtctggcctcccagcatggtaccacggacctgtttagcacgctggaacactatcgtaaagtgttcctgccgaataccagtaacaatgattggtttaaatccgaaacgaaagcgtatattgtggaagaaaaaagcaccatcgaagaagttaaaacgaaacagggtctggcgggcaccaaatacagtattggcgtttatgatcgcatcaccagcgccacgtggaaatatcgcaacatggtgctgccgctgctgaccctgccggaacgctctgtgttcgttattagtacgatgtcctcactgggttttggcgcctacgaccgttatcgctcgagcgatcataaagcgggtaaagccctgaatgattttgtggaagaaaacgctcgtgaaaccgcgaaacgtcagcgcgaccactatgattactggtatcgcattctggatgacaatgcgcgtgaaaaactgtatcgcaacatcctgctgtacgatgcctataaattcggcgatgacaataccgtgggtaaagccacggaagttgcagattttgacaatccgaacccggcgatgcaacatttctttggtccggtcggcaataaagtgggtcataaccagcacggcgcgtatgcgaccggtgatgcagtgtattacatgggctaccgtatgctggataaagacggtgctattacctatacgcatgaaatgacccacgatagtgaccaggatatctacctgggcggttatggtcgtcgctccggtctgggcccggaatttttcgctaaaggtctgctgcaggcgccggatcatccggatgacgcaaccattacgatcaattcaattctgaaacactcgaaaagcgactctaccgaatcgcgtcgcctgcaagttctggatccgaccacgcgcttcaacaatgcggatgacctgaaacagtatgtgcataacatgtttgatgttgtctacatgctggaatatctggaaggcaatagcattctgaaactggacaccaaccagaaacagcaactgctgcgtaaagttacgaatgaatatcacccggacccggatggtaacaaagtgtacgcgaccaatgtggttcgcaacctgacggtcgaagaagtggaacgtctgcgctcattcaacgacctgattgataacaatatcctgtctagtcgtgaatacgcatcgggcaaatatgaacgcaatggttactttaccattaaactgttcgctccgatctacgcagctctgagtaacgacattggtacgccgggtgatctgatgggtcgtcgcatcgcctatgaactgctggcggccaaaggctttaaagatggtatggttccgtatattagcaatcagtacgaagaagaagcgaaacaaaaaggtaaaaccatcaacctgtatggcaaaacccgtggtctggtgacggatgacctggttctggaaaaagtcttcaacaatcaataccatacctggagcgaatttaaaaaagcgatgtatcaggaacgtcaggaccaatttgatcgcctgaataaagttaccttcaacgataccacgcagccgtggcaaacgtttgcgaagaaaaccacgtcctcagtggatgaactgcagaaactgatggacgtcgccgtgcgtaaagatgcagaacataactactaccactggaacaactacaacccggacattgatagcgaagtgcacaaactgaaacgcgcgatcttcaaagcgtacctggaccaaaccaatgacttccgttctagtatcttcgaaaacaaaaaa

SEQ ID NO: 10 - DNA, 4713 bp, synthetic construct
  source 1..4713: mol_type = other DNA
acatgcccaccgtgcccagcacctgaactcctggggggaccgtcagtcttcctcttccccccaaaacccaaggacaccctcatgatctcccggacccctgaggtcacatgcgtggtggtggacgtgagccacgaagaccctgaggtcaagttcaactggtacgtggacggcgtggaggtgcataatgccaagacaaagccgcgggaggagcagtacaacagcacgtaccgggtggtcagcgtcctcaccgtcctgcaccaggactggctgaatggcaaggagtacaagtgcaaggtctccaacaaagccctcccagcccccatcgagaaaaccatctccaaagccaaagggcagccccgagaaccacaggtgtacaccctgcccccatcccgggatgagctgaccaagaaccaggtcagcctgacctgcctggtcaaaggcttctatcccagcgacatcgccgtggagtgggagagcaatgggcagccggagaacaactacaagaccacgcctcccgtgctggactccgacggctccttcttcctctacagcaagctcaccgtggacaagagcaggtggcagcaggggaacgtcttctcatgctccgtgatgcatgaggctctgcacaaccactacacgcagaagagcctctccctgtctccgggtaaaggtggcggtggcggcggttctagaggcaacaccacgagcgaaaacggtcagaccgaaccggaaccgtccaacggcaattcaacggaagatgttagtaccgaatccaatacgtctaacagtaacggtaacgaagaaatcaaacaggaaaacgaactggatccggacaaaaaagtcgaagaaccggaaaaaaccctggaactgcgcaatgtgagcgatctggaactgtattccctgtcaaacggcacgtacaaacagcatatctctctggaacaagttccgtcgaatccgaacagctactttgttaaagtcaaatcatcgagcttcaaagatgtgtatctgccggttgcatcgatcagcgaagaacgtaaaaatgacaaaatcctgtacaaaatcaccgctaaagtggaaaaactgcagcaagaaatcgaaagccgctataaagataactttacgttctacctggcgaaaaaaggtaccgaagaaaccacgaattttacgtctttcagtaacctggttaaagcgattaatcagaacccgtcaggcacctaccacctggcagcttcgctgaatgccaacgaagtggaactgggtccggacgaacgtagctatattaaagataccttcacgggtcgcctgatcggcgaaaaagatggtaaaaactacgccatctacaacctgaaaaaaccgctgtttgaaaatctgtctggcgcgaccgttgaaaaactgtcgctgaaaaacgtcgccattagcggtaaagatgacatcggctctctggcgaatgaagcccagaacaataccaaaatcaaacaagtgcatgttgatggcgtgctggcaggtgaacgtggcattggcggtctgctggcgaaagccgaacagtctagtatcaccgaatcctcatttaaaggtcgcattatcaatacgtatgaaaccacggcggcctacaacattggcggtatggttggccacctgaccggtgataaagccctgctgaccaaaagcaaagcaacggtggctatctcgagcaataccaacacgtctgatcagaccgttggcggtctggctggtctggtcgatcgtgacgcgcagattcaagactcttatgccgaaggcgatatcaacaatgttaaacattttggtcgcgtggcgggtgttgccggcaatctgtgggaccgtaccagtggcgatgttcgccacgcaggttcgctgacgaatgtcctgagcgatgtcaacgtgaccaatggtaacgctattacgggctaccattacaacgaaatgaaagtgaaagataccttctctagtaaagcgaatcgtgtctataacgtgacgctggttaaagatgaagtcgtgtcaaaagaatcgtttgaagaacgcggcaccatgctggacgcatctcagatcgctagtaaaaaagcggaaattaacccgctgatcctgccgaccgttgaaccgctgtccacgtcaggtaaaaaagatagcgacttctctaaagtggcctattaccaggcaaaacgtaacctgacctacaaaaacatcgaaaaactgctgccgttctacaacaaagccacgatcgtcaaatacggcaacctggtgaatgaaaacagcctgctgtatcagaaagaactgctgtctgcggtgatgatgaaagacaatcaggtcattaccgatatcgtgagtaataaacaaacggccaacaaactgctgctgcattataaagatgacctgtccgaaaaactggacctgaaatatcagaacgatttcgcaaaactggctgaatactcactgggtaataccggcctgctgtatacgccgaaccagtttctgtacgatcaaacctcgattatcaaacaggtgctgccggacctgcaaaaagttgattaccactcagaagcaattcgcaaaaccctgggtatctcgccgaatgtgaaacagacggaactgtatctggaagatcaatttgctaaaaccaaacagcaactggaagactctctgaaaaaactgctgagtgcagatgctggcctggcgtctgccaatccggttaccgaaggttacctggtcgataaaattaaacgtaacaaagaagccctgctgctgggcctgacctatctggaacgctggtacaatttcagctatggtcaggttaacgtcaaagacctggtgctgtatcatctggatttctttggtaaaggcaacgcaagtccgctggataccctgattgaactgggtaaatccggctttaacaatctgctggcgaaaaacaatgttgacacctacggcatcagtctggcctcccagcatggtaccacggacctgtttagcacgctggaacactatcgtaaagtgttcctgccgaataccagtaacaatgattggtttaaatccgaaacgaaagcgtatattgtggaagaaaaaagcaccatcgaagaagttaaaacgaaacagggtctggcgggcaccaaatacagtattggcgtttatgatcgcatcaccagcgccacgtggaaatatcgcaacatggtgctgccgctgctgaccctgccggaacgctctgtgttcgttattagtacgatgtcctcactgggttttggcgcctacgaccgttatcgctcgagcgatcataaagcgggtaaagccctgaatgattttgtggaagaaaacgctcgtgaaaccgcgaaacgtcagcgcgaccactatgattactggtatcgcattctggatgacaatgcgcgtgaaaaactgtatcgcaacatcctgctgtacgatgcctataaattcggcgatgacaataccgtgggtaaagccacggaagttgcagattttgacaatccgaacccggcgatgcaacatttctttggtccggtcggcaataaagtgggtcataaccagcacggcgcgtatgcgaccggtgatgcagtgtattacatgggctaccgtatgctggataaagacggtgctattacctatacgcatgaaatgacccacgatagtgaccaggatatctacctgggcggttatggtcgtcgctccggtctgggcccggaatttttcgctaaaggtctgctgcaggcgccggatcatccggatgacgcaaccattacgatcaattcaattctgaaacactcgaaaagcgactctaccgaatcgcgtcgcctgcaagttctggatccgaccacgcgcttcaacaatgcggatgacctgaaacagtatgtgcataacatgtttgatgttgtctacatgctggaatatctggaaggcaatagcattctgaaactggacaccaaccagaaacagcaactgctgcgtaaagttacgaatgaatatcacccggacccggatggtaacaaagtgtacgcgaccaatgtggttcgcaacctgacggtcgaagaagtggaacgtctgcgctcattcaacgacctgattgataacaatatcctgtctagtcgtgaatacgcatcgggcaaatatgaacgcaatggttactttaccattaaactgttcgctccgatctacgcagctctgagtaacgacattggtacgccgggtgatctgatgggtcgtcgcatcgcctatgaactgctggcggccaaaggctttaaagatggtatggttccgtatattagcaatcagtacgaagaagaagcgaaacaaaaaggtaaaaccatcaacctgtatggcaaaacccgtggtctggtgacggatgacctggttctggaaaaagtcttcaacaatcaataccatacctggagcgaatttaaaaaagcgatgtatcaggaacgtcaggaccaatttgatcgcctgaataaagttaccttcaacgataccacgcagccgtggcaaacgtttgcgaagaaaaccacgtcctcagtggatgaactgcagaaactgatggacgtcgccgtgcgtaaagatgcagaacataactactaccactggaacaactacaacccggacattgatagcgaagtgcacaaactgaaacgcgcgatcttcaaagcgtacctggaccaaaccaatgacttccgttctagtatcttcgaaaacaaaaaa

SEQ ID NO: 11 - DNA, 4740 bp, synthetic construct
  source 1..4740: mol_type = other DNA
ggcaacaccacgagcgaaaacggtcagaccgaaccggaaccgtccaacggcaattcaacggaagatgttagtaccgaatccaatacgtctaacagtaacggtaacgaagaaatcaaacaggaaaacgaactggatccggacaaaaaagtcgaagaaccggaaaaaaccctggaactgcgcaatgtgagcgatctggaactgtattccctgtcaaacggcacgtacaaacagcatatctctctggaacaagttccgtcgaatccgaacagctactttgttaaagtcaaatcatcgagcttcaaagatgtgtatctgccggttgcatcgatcagcgaagaacgtaaaaatgacaaaatcctgtacaaaatcaccgctaaagtggaaaaactgcagcaagaaatcgaaagccgctataaagataactttacgttctacctggcgaaaaaaggtaccgaagaaaccacgaattttacgtctttcagtaacctggttaaagcgattaatcagaacccgtcaggcacctaccacctggcagcttcgctgaatgccaacgaagtggaactgggtccggacgaacgtagctatattaaagataccttcacgggtcgcctgatcggcgaaaaagatggtaaaaactacgccatctacaacctgaaaaaaccgctgtttgaaaatctgtctggcgcgaccgttgaaaaactgtcgctgaaaaacgtcgccattagcggtaaagatgacatcggctctctggcgaatgaagcccagaacaataccaaaatcaaacaagtgcatgttgatggcgtgctggcaggtgaacgtggcattggcggtctgctggcgaaagccgaacagtctagtatcaccgaatcctcatttaaaggtcgcattatcaatacgtatgaaaccacggcggcctacaacattggcggtatggttggccacctgaccggtgataaagccctgctgaccaaaagcaaagcaacggtggctatctcgagcaataccaacacgtctgatcagaccgttggcggtctggctggtctggtcgatcgtgacgcgcagattcaagactcttatgccgaaggcgatatcaacaatgttaaacattttggtcgcgtggcgggtgttgccggcaatctgtgggaccgtaccagtggcgatgttcgccacgcaggttcgctgacgaatgtcctgagcgatgtcaacgtgaccaatggtaacgctattacgggctaccattacaacgaaatgaaagtgaaagataccttctctagtaaagcgaatcgtgtctataacgtgacgctggttaaagatgaagtcgtgtcaaaagaatcgtttgaagaacgcggcaccatgctggacgcatctcagatcgctagtaaaaaagcggaaattaacccgctgatcctgccgaccgttgaaccgctgtccacgtcaggtaaaaaagatagcgacttctctaaagtggcctattaccaggcaaaacgtaacctgacctacaaaaacatcgaaaaactgctgccgttctacaacaaagccacgatcgtcaaatacggcaacctggtgaatgaaaacagcctgctgtatcagaaagaactgctgtctgcggtgatgatgaaagacaatcaggtcattaccgatatcgtgagtaataaacaaacggccaacaaactgctgctgcattataaagatgacctgtccgaaaaactggacctgaaatatcagaacgatttcgcaaaactggctgaatactcactgggtaataccggcctgctgtatacgccgaaccagtttctgtacgatcaaacctcgattatcaaacaggtgctgccggacctgcaaaaagttgattaccactcagaagcaattcgcaaaaccctgggtatctcgccgaatgtgaaacagacggaactgtatctggaagatcaatttgctaaaaccaaacagcaactggaagactctctgaaaaaactgctgagtgcagatgctggcctggcgtctgccaatccggttaccgaaggttacctggtcgataaaattaaacgtaacaaagaagccctgctgctgggcctgacctatctggaacgctggtacaatttcagctatggtcaggttaacgtcaaagacctggtgctgtatcatctggatttctttggtaaaggcaacgcaagtccgctggataccctgattgaactgggtaaatccggctttaacaatctgctggcgaaaaacaatgttgacacctacggcatcagtctggcctcccagcatggtaccacggacctgtttagcacgctggaacactatcgtaaagtgttcctgccgaataccagtaacaatgattggtttaaatccgaaacgaaagcgtatattgtggaagaaaaaagcaccatcgaagaagttaaaacgaaacagggtctggcgggcaccaaatacagtattggcgtttatgatcgcatcaccagcgccacgtggaaatatcgcaacatggtgctgccgctgctgaccctgccggaacgctctgtgttcgttattagtacgatgtcctcactgggttttggcgcctacgaccgttatcgctcgagcgatcataaagcgggtaaagccctgaatgattttgtggaagaaaacgctcgtgaaaccgcgaaacgtcagcgcgaccactatgattactggtatcgcattctggatgacaatgcgcgtgaaaaactgtatcgcaacatcctgctgtacgatgcctataaattcggcgatgacaataccgtgggtaaagccacggaagttgcagattttgacaatccgaacccggcgatgcaacatttctttggtccggtcggcaataaagtgggtcataaccagcacggcgcgtatgcgaccggtgatgcagtgtattacatgggctaccgtatgctggataaagacggtgctattacctatacgcatgaaatgacccacgatagtgaccaggatatctacctgggcggttatggtcgtcgctccggtctgggcccggaatttttcgctaaaggtctgctgcaggcgccggatcatccggatgacgcaaccattacgatcaattcaattctgaaacactcgaaaagcgactctaccgaatcgcgtcgcctgcaagttctggatccgaccacgcgcttcaacaatgcggatgacctgaaacagtatgtgcataacatgtttgatgttgtctacatgctggaatatctggaaggcaatagcattctgaaactggacaccaaccagaaacagcaactgctgcgtaaagttacgaatgaatatcacccggacccggatggtaacaaagtgtacgcgaccaatgtggttcgcaacctgacggtcgaagaagtggaacgtctgcgctcattcaacgacctgattgataacaatatcctgtctagtcgtgaatacgcatcgggcaaatatgaacgcaatggttactttaccattaaactgttcgctccgatctacgcagctctgagtaacgacattggtacgccgggtgatctgatgggtcgtcgcatcgcctatgaactgctggcggccaaaggctttaaagatggtatggttccgtatattagcaatcagtacgaagaagaagcgaaacaaaaaggtaaaaccatcaacctgtatggcaaaacccgtggtctggtgacggatgacctggttctggaaaaagtcttcaacaatcaataccatacctggagcgaatttaaaaaagcgatgtatcaggaacgtcaggaccaatttgatcgcctgaataaagttaccttcaacgataccacgcagccgtggcaaacgtttgcgaagaaaaccacgtcctcagtggatgaactgcagaaactgatggacgtcgccgtgcgtaaagatgcagaacataactactaccactggaacaactacaacccggacattgatagcgaagtgcacaaactgaaacgcgcgatcttcaaagcgtacctggaccaaaccaatgacttccgttctagtatcttcgaaaacaaaaaaagatctggtggcggtggctctcaccatcatcaccaccatcatcatcaccacacatgcccaccgtgcccagcacctgaactcctggggggaccgtcagtcttcctcttccccccaaaacccaaggacaccctcatgatctcccggacccctgaggtcacatgcgtggtggtggacgtgagccacgaagaccctgaggtcaagttcaactggtacgtggacggcgtggaggtgcataatgccaagacaaagccgcgggaggagcagtacaacagcacgtaccgggtggtcagcgtcctcaccgtcctgcaccaggactggctgaatggcaaggagtacaagtgcaaggtctccaacaaagccctcccagcccccatcgagaaaaccatctccaaagccaaagggcagccccgagaaccacaggtgtacaccctgcccccatcccgggatgagctgaccaagaaccaggtcagcctgacctgcctggtcaaaggcttctatcccagcgacatcgccgtggagtgggagagcaatgggcagccggagaacaactacaagaccacgcctcccgtgctggactccgacggctccttcttcctctacagcaagctcaccgtggacaagagcaggtggcagcaggggaacgtcttctcatgctccgtgatgcatgaggctctgcacaaccactacacgcagaagagcctctccctgtctccgggtaaa

SEQ ID NO: 12 - DNA, 4728 bp, synthetic construct
  source 1..4728: mol_type = other DNA
ggcaacaccacgagcgaaaacggtcagaccgaaccggaaccgtccaacggcaattcaacggaagatgttagtaccgaatccaatacgtctaacagtaacggtaacgaagaaatcaaacaggaaaacgaactggatccggacaaaaaagtcgaagaaccggaaaaaaccctggaactgcgcaatgtgagcgatctggaactgtattccctgtcaaacggcacgtacaaacagcatatctctctggaacaagttccgtcgaatccgaacagctactttgttaaagtcaaatcatcgagcttcaaagatgtgtatctgccggttgcatcgatcagcgaagaacgtaaaaatgacaaaatcctgtacaaaatcaccgctaaagtggaaaaactgcagcaagaaatcgaaagccgctataaagataactttacgttctacctggcgaaaaaaggtaccgaagaaaccacgaattttacgtctttcagtaacctggttaaagcgattaatcagaacccgtcaggcacctaccacctggcagcttcgctgaatgccaacgaagtggaactgggtccggacgaacgtagctatattaaagataccttcacgggtcgcctgatcggcgaaaaagatggtaaaaactacgccatctacaacctgaaaaaaccgctgtttgaaaatctgtctggcgcgaccgttgaaaaactgtcgctgaaaaacgtcgccattagcggtaaagatgacatcggctctctggcgaatgaagcccagaacaataccaaaatcaaacaagtgcatgttgatggcgtgctggcaggtgaacgtggcattggcggtctgctggcgaaagccgaacagtctagtatcaccgaatcctcatttaaaggtcgcattatcaatacgtatgaaaccacggcggcctacaacattggcggtatggttggccacctgaccggtgataaagccctgctgaccaaaagcaaagcaacggtggctatctcgagcaataccaacacgtctgatcagaccgttggcggtctggctggtctggtcgatcgtgacgcgcagattcaagactcttatgccgaaggcgatatcaacaatgttaaacattttggtcgcgtggcgggtgttgccggcaatctgtgggaccgtaccagtggcgatgttcgccacgcaggttcgctgacgaatgtcctgagcgatgtcaacgtgaccaatggtaacgctattacgggctaccattacaacgaaatgaaagtgaaagataccttctctagtaaagcgaatcgtgtctataacgtgacgctggttaaagatgaagtcgtgtcaaaagaatcgtttgaagaacgcggcaccatgctggacgcatctcagatcgctagtaaaaaagcggaaattaacccgctgatcctgccgaccgttgaaccgctgtccacgtcaggtaaaaaagatagcgacttctctaaagtggcctattaccaggcaaaacgtaacctgacctacaaaaacatcgaaaaactgctgccgttctacaacaaagccacgatcgtcaaatacggcaacctggtgaatgaaaacagcctgctgtatcagaaagaactgctgtctgcggtgatgatgaaagacaatcaggtcattaccgatatcgtgagtaataaacaaacggccaacaaactgctgctgcattataaagatgacctgtccgaaaaactggacctgaaatatcagaacgatttcgcaaaactggctgaatactcactgggtaataccggcctgctgtatacgccgaaccagtttctgtacgatcaaacctcgattatcaaacaggtgctgccggacctgcaaaaagttgattaccactcagaagcaattcgcaaaaccctgggtatctcgccgaatgtgaaacagacggaactgtatctggaagatcaatttgctaaaaccaaacagcaactggaagactctctgaaaaaactgctgagtgcagatgctggcctggcgtctgccaatccggttaccgaaggttacctggtcgataaaattaaacgtaacaaagaagccctgctgctgggcctgacctatctggaacgctggtacaatttcagctatggtcaggttaacgtcaaagacctggtgctgtatcatctggatttctttggtaaaggcaacgcaagtccgctggataccctgattgaactgggtaaatccggctttaacaatctgctggcgaaaaacaatgttgacacctacggcatcagtctggcctcccagcatggtaccacggacctgtttagcacgctggaacactatcgtaaagtgttcctgccgaataccagtaacaatgattggtttaaatccgaaacgaaagcgtatattgtggaagaaaaaagcaccatcgaagaagttaaaacgaaacagggtctggcgggcaccaaatacagtattggcgtttatgatcgcatcaccagcgccacgtggaaatatcgcaacatggtgctgccgctgctgaccctgccggaacgctctgtgttcgttattagtacgatgtcctcactgggttttggcgcctacgaccgttatcgctcgagcgatcataaagcgggtaaagccctgaatgattttgtggaagaaaacgctcgtgaaaccgcgaaacgtcagcgcgaccactatgattactggtatcgcattctggatgacaatgcgcgtgaaaaactgtatcgcaacatcctgctgtacgatgcctataaattcggcgatgacaataccgtgggtaaagccacggaagttgcagattttgacaatccgaacccggcgatgcaacatttctttggtccggtcggcaataaagtgggtcataaccagcacggcgcgtatgcgaccggtgatgcagtgtattacatgggctaccgtatgctggataaagacggtgctattacctatacgcatgaaatgacccacgatagtgaccaggatatctacctgggcggttatggtcgtcgctccggtctgggcccggaatttttcgctaaaggtctgctgcaggcgccggatcatccggatgacgcaaccattacgatcaattcaattctgaaacactcgaaaagcgactctaccgaatcgcgtcgcctgcaagttctggatccgaccacgcgcttcaacaatgcggatgacctgaaacagtatgtgcataacatgtttgatgttgtctacatgctggaatatctggaaggcaatagcattctgaaactggacaccaaccagaaacagcaactgctgcgtaaagttacgaatgaatatcacccggacccggatggtaacaaagtgtacgcgaccaatgtggttcgcaacctgacggtcgaagaagtggaacgtctgcgctcattcaacgacctgattgataacaatatcctgtctagtcgtgaatacgcatcgggcaaatatgaacgcaatggttactttaccattaaactgttcgctccgatctacgcagctctgagtaacgacattggtacgccgggtgatctgatgggtcgtcgcatcgcctatgaactgctggcggccaaaggctttaaagatggtatggttccgtatattagcaatcagtacgaagaagaagcgaaacaaaaaggtaaaaccatcaacctgtatggcaaaacccgtggtctggtgacggatgacctggttctggaaaaagtcttcaacaatcaataccatacctggagcgaatttaaaaaagcgatgtatcaggaacgtcaggaccaatttgatcgcctgaataaagttaccttcaacgataccacgcagccgtggcaaacgtttgcgaagaaaaccacgtcctcagtggatgaactgcagaaactgatggacgtcgccgtgcgtaaagatgcagaacataactactaccactggaacaactacaacccggacattgatagcgaagtgcacaaactgaaacgcgcgatcttcaaagcgtacctggaccaaaccaatgacttccgttctagtatcttcgaaaacaaaaaaagatctggcggtggtggtagcgaatcgaagtacggtccgccgtgtccgagttgcccggctccggagtttctgggtggccctagcgtgttcttatttccgccaaagccgaaggacaccctgatgatcagccgcaccccggaggtaacttgcgtcgtcgtggatgtttcccaagaagatccggaggtgcagtttaactggtatgtggacggcgttgaagttcataatgcgaaaaccaagccgcgtgaagagcagttcaacagcacctatcgtgtggtctccgtgttgacggttcttcaccaggattggttgaatggtaaagaatataagtgcaaagtttccaataaaggcctgccgtcgagcattgaaaaaacgattagcaaggcaaagggccaacctcgcgagccgcaagtgtacactctgccgccgagccaagaggaaatgaccaaaaaccaggtttcattgacctgcctggttaagggtttttacccgagcgacatcgccgttgagtgggaatctaacggccagccggagaacaactacaagaccaccccaccggttctggacagcgatggttccttcttcctgtactcccgtctcaccgtggacaaaagccgttggcaagagggaaacgtgttctcttgtagcgtgatgcatgaagcgctgcacaatcattatacgcagaaatctctgagcctttctctgggcaaa

SEQ ID NO: 13 - protein, 223 aa, synthetic construct
TCPPCPAPELLGGPSVFLFPPKPKDTLMISRTPEVTCVVVDVSHEDPEVKFNWYVDGVEVHNAKTKPREEQYNSTYRVVSVLTVLHQDWLNGKEYKCKVSNKALPAPIEKTISKAKGQPREPQVYTLPPSRDELTKNQVSLTCLVKGFYPSDIAVEWESNGQPENNYKTTPPVLDSDGSFFLYSKLTVDKSRWQQGNVFSCSVMHEALHNHYTQKSLSLSPGK

SEQ ID NO: 14 - protein, 229 aa, synthetic construct
ESKYGPPCPSCPAPEFLGGPSVFLFPPKPKDTLMISRTPEVTCVVVDVSQEDPEVQFNWYVDGVEVHNAKTKPREEQFNSTYRVVSVLTVLHQDWLNGKEYKCKVSNKGLPSSIEKTISKAKGQPREPQVYTLPPSQEEMTKNQVSLTCLVKGFYPSDIAVEWESNGQPENNYKTTPPVLDSDGSFFLYSRLTVDKSRWQEGNVFSCSVMHEALHNHYTQKSLSLSLGK

SEQ ID NO: 15 - protein, 4 aa, synthetic construct
GGGS

SEQ ID NO: 16 - protein, 5 aa, synthetic construct
GGGGS

SEQ ID NO: 17 - protein, 7 aa, synthetic construct
GGGGGGS

SEQ ID NO: 18 - protein, 15 aa, synthetic construct
GGGGSGGGGSGGGGS

SEQ ID NO: 19 - skipped

SEQ ID NO: 20 - protein, 7 aa, synthetic construct
GSSGSSG

SEQ ID NO: 21 - protein, 9 aa, synthetic construct
RSGSSGSSG

SEQ ID NO: 22 - protein, 1962 aa, synthetic construct
QETAGVHYKYVADSELSSEEKKQLVYDIPTYVENDDETYYLVYKLNSQNQLAELPNTGSKNERQALVAGASLAAMGILIFAVSKKKVKNKTVLHLVLVAGIGNGVLVSVHALENHLLLNYNTDYELTSGEKLPLPKEISGYTYIGYIKEGKTTSESEVSNQKSSVATPTKQQKVDYNVTPNFVDHPSTVQAIQEQTPVSSTKPTEVQVVEKPFSTELINPRKEEKQSSDSQEQLAEHKNLETKKEEKISPKEKTGVNTLNPQDEVLSGQLNKPELLYREETMETKIDFQEEIQENPDLAEGTVRVKQEGKLGKKVEIVRIFSVNKEEVSREIVSTSTTAPSPRIVEKGTKKTQVIKEQPETGVEHKDVQSGAIVEPAIQPELPEAVVSDKGEPEVQPTLPEAVVTDKGETEVQPESPDTVVSDKGEPEQVAPLPEYKGNIEQVKPETPVEKTKEQGPEKTEEVPVKPTEETPVNPNEGTTEGTSIQEAENPVQPAEESTTNSEKVSPDTSSKNTGEVSSNPSDSTTSVGESNKPEHNDSKNENSEKTVEEVPVNPNEGTVEGTSNQETEKPVQPAEETQTNSGKIANENTGEVSNKPSDSKPPVEESNQPEKNGTATKPENSGNTTSENGQTEPEPSNGNSTEDVSTESNTSNSNGNEEIKQENELDPDKKVEEPEKTLELRNVSDLELYSLSNGTYKQHISLEQVPSNPNSYFVKVKSSSFKDVYLPVASISEERKNDKILYKITAKVEKLQQEIESRYKDNFTFYLAKKGTEETTNFTSFSNLVKAINQNPSGTYHLAASLNANEVELGPDERSYIKDTFTGRLIGEKDGKNYAIYNLKKPLFENLSGATVEKLSLKNVAISGKDDIGSLANEAQNNTKIKQVHVDGVLAGERGIGGLLAKAEQSSITESSFKGRIINTYETTAAYNIGGMVGHLTGDKALLTKSKATVAISSNTNTSDQTVGGLAGLVDRDAQIQDSYAEGDINNVKHFGRVAGVAGNLWDRTSGDVRHAGSLTNVLSDVNVTNGNAITGYHYNEMKVKDTFSSKANRVYNVTLVKDEVVSKESFEERGTMLDASQIASKKAEINPLILPTVEPLSTSGKKDSDFSKVAYYQAKRNLTYKNIEKLLPFYNKATIVKYGNLVNENSLLYQKELLSAVMMKDNQVITDIVSNKQTANKLLLHYKDDLSEKLDLKYQNDFAKLAEYSLGNTGLLYTPNQFLYDQTSIIKQVLPDLQKVDYHSEAIRKTLGISPNVKQTELYLEDQFAKTKQQLEDSLKKLLSADAGLASANPVTEGYLVDKIKRNKEALLLGLTYLERWYNFSYGQVNVKDLVLYHLDFFGKGNASPLDTLIELGKSGFNNLLAKNNVDTYGISLASQHGTTDLFSTLEHYRKVFLPNTSNNDWFKSETKAYIVEEKSTIEEVKTKQGLAGTKYSIGVYDRITSATWKYRNMVLPLLTLPERSVFVISTMSSLGFGAYDRYRSSDHKAGKALNDFVEENARETAKRQRDHYDYWYRILDDNAREKLYRNILLYDAYKFGDDNTVGKATEVADFDNPNPAMQHFFGPVGNKVGHNQHGAYATGDAVYYMGYRMLDKDGAITYTHEMTHDSDQDIYLGGYGRRSGLGPEFFAKGLLQAPDHPDDATITINSILKHSKSDSTESRRLQVLDPTTRFNNADDLKQYVHNMFDVVYMLEYLEGNSILKLDTNQKQQLLRKVTNEYHPDPDGNKVYATNVVRNLTVEEVERLRSFNDLIDNNILSSREYASGKYERNGYFTIKLFAPIYAALSNDIGTPGDLMGRRIAYELLAAKGFKDGMVPYISNQYEEEAKQKGKTINLYGKTRGLVTDDLVLEKVFNNQYHTWSEFKKAMYQERQDQFDRLNKVTFNDTTQPWQTFAKKTTSSVDELQKLMDVAVRKDAEHNYYHWNNYNPDIDSEVHKLKRAIFKAYLDQTNDFRSSIFENKK

SEQ ID NO: 23 - protein, 585 aa, synthetic construct [sequence omitted]

SEQ ID NO: 24 - protein, 1578 aa, synthetic construct
GNTTSENGQTEPEPSNGNSTEDVSTESNTSNSNGNEEIKQENELDPDKKVEEPEKTLELRNVSDLELYSLSNGTYKQHISLEQVPSNPNSYFVKVKSSSFKDVYLPVASISEERKNDKILYKITAKVEKLQQEIESRYKDNFTFYLAKKGTEETTNFTSFSNLVKAINQNPSGTYHLAASLNANEVELGPDERSYIKDTFTGRLIGEKDGKNYAIYNLKKPLFENLSGATVEKLSLKNVAISGKDDIGSLANEAQNNTKIKQVHVDGVLAGERGIGGLLAKAEQSSITESSFKGRIINTYETTAAYNIGGMVGHLTGDKALLTKSKATVAISSNTNTSDQTVGGLAGLVDRDAQIQDSYAEGDINNVKHFGRVAGVAGNLWDRTSGDVRHAGSLTNVLSDVNVTNGNAITGYHYNEMKVKDTFSSKANRVYNVTLVKDEVVSKESFEERGTMLDASQIASKKAEINPLILPTVEPLSTSGKKDSDFSKVAYYQAKRNLTYKNIEKLLPFYNKATIVKYGNLVNENSLLYQKELLSAVMMKDNQVITDIVSNKQTANKLLLHYKDDLSEKLDLKYQNDFAKLAEYSLGNTGLLYTPNQFLYDQTSIIKQVLPDLQKVDYHSEAIRKTLGISPNVKQTELYLEDQFAKTKQQLEDSLKKLLSADAGLASANPVTEGYLVDKIKRNKEALLLGLTYLERWYNFSYGQVNVKDLVLYHLDFFGKGNASPLDTLIELGKSGFNNLLAKNNVDTYGISLASQHGTTDLFSTLEHYRKVFLPNTSNNDWFKSETKAYIVEEKSTIEEVKTKQGLAGTKYSIGVYDRITSATWKYRNMVLPLLTLPERSVFVISTMSSLGFGAYDRYRSSDHKAGKALNDFVEENARETAKRQRDHYDYWYRILDDNAREKLYRNILLYDAYKFGDDNTVGKATEVADFDNPNPAMQHFFGPVGNKVGHNQHGAYATGDAVYYMGYRMLDKDGAITYTHEMTHDSDQDIYLGGYGRRSGLGPEFFAKGLLQAPDHPDDATITINSILKHSKSDSTESRRLQVLDPTTRFNNADDLKQYVHNMFDVVYMLEYLEGNSILKLDTNQKQQLLRKVTNEYHPDPDGNKVYATNVVRNLTVEEVERLRSFNDLIDNNILSSREYASGKYERNGYFTIKLFAPIYAALSNDIGTPGDLMGRRIAYELLAAKGFKDGMVPYISNQYEEEAKQKGKTINLYGKTRGLVTDDLVLEKVFNNQYHTWSEFKKAMYQERQDQFDRLNKVTFNDTTQPWQTFAKKTTSSVDELQKLMDVAVRKDAEHNYYHWNNYNPDIDSEVHKLKRAIFKAYLDQTNDFRSSIFENKKRSGSSGSSGESKYGPPCPSCPAPEFLGGPSVFLFPPKPKDTLMISRTPEVTCVVVDVSQEDPEVQFNWYVDGVEVHNAKTKPREEQFNSTYRVVSVLTVLHQDWLNGKEYKCKVSNKGLPSSIEKTISKAKGQPREPQVYTLPPSQEEMTKNQVSLTCLVKGFYPSDIAVEWESNGQPENNYKTTPPVLDSDGSFFLYSRLTVDKSRWQEGNVFSCSVMHEALHNHYTQKSLSLSLGK

SEQ ID NO: 25 - DNA, 4740 bp, synthetic construct
  source 1..4740: mol_type = other DNA
ggcaacaccacgagcgaaaacggtcagaccgaaccggaaccgtccaacggcaattcaacggaagatgttagtaccgaatccaatacgtctaacagtaacggtaacgaagaaatcaaacaggaaaacgaactggatccggacaaaaaagtcgaagaaccggaaaaaaccctggaactgcgcaatgtgagcgatctggaactgtattccctgtcaaacggcacgtacaaacagcatatctctctggaacaagttccgtcgaatccgaacagctactttgttaaagtcaaatcatcgagcttcaaagatgtgtatctgccggttgcatcgatcagcgaagaacgtaaaaatgacaaaatcctgtacaaaatcaccgctaaagtggaaaaactgcagcaagaaatcgaaagccgctataaagataactttacgttctacctggcgaaaaaaggtaccgaagaaaccacgaattttacgtctttcagtaacctggttaaagcgattaatcagaacccgtcaggcacctaccacctggcagcttcgctgaatgccaacgaagtggaactgggtccggacgaacgtagctatattaaagataccttcacgggtcgcctgatcggcgaaaaagatggtaaaaactacgccatctacaacctgaaaaaaccgctgtttgaaaatctgtctggcgcgaccgttgaaaaactgtcgctgaaaaacgtcgccattagcggtaaagatgacatcggctctctggcgaatgaagcccagaacaataccaaaatcaaacaagtgcatgttgatggcgtgctggcaggtgaacgtggcattggcggtctgctggcgaaagccgaacagtctagtatcaccgaatcctcatttaaaggtcgcattatcaatacgtatgaaaccacggcggcctacaacattggcggtatggttggccacctgaccggtgataaagccctgctgaccaaaagcaaagcaacggtggctatctcgagcaataccaacacgtctgatcagaccgttggcggtctggctggtctggtcgatcgtgacgcgcagattcaagactcttatgccgaaggcgatatcaacaatgttaaacattttggtcgcgtggcgggtgttgccggcaatctgtgggaccgtaccagtggcgatgttcgccacgcaggttcgctgacgaatgtcctgagcgatgtcaacgtgaccaatggtaacgctattacgggctaccattacaacgaaatgaaagtgaaagataccttctctagtaaagcgaatcgtgtctataacgtgacgctggttaaagatgaagtcgtgtcaaaagaatcgtttgaagaacgcggcaccatgctggacgcatctcagatcgctagtaaaaaagcggaaattaacccgctgatcctgccgaccgttgaaccgctgtccacgtcaggtaaaaaagatagcgacttctctaaagtggcctattaccaggcaaaacgtaacctgacctacaaaaacatcgaaaaactgctgccgttctacaacaaagccacgatcgtcaaatacggcaacctggtgaatgaaaacagcctgctgtatcagaaagaactgctgtctgcggtgatgatgaaagacaatcaggtcattaccgatatcgtgagtaataaacaaacggccaacaaactgctgctgcattataaagatgacctgtccgaaaaactggacctgaaatatcagaacgatttcgcaaaactggctgaatactcactgggtaataccggcctgctgtatacgccgaaccagtttctgtacgatcaaacctcgattatcaaacaggtgctgccggacctgcaaaaagttgattaccactcagaagcaattcgcaaaaccctgggtatctcgccgaatgtgaaacagacggaactgtatctggaagatcaatttgctaaaaccaaacagcaactggaagactctctgaaaaaactgctgagtgcagatgctggcctggcgtctgccaatccggttaccgaaggttacctggtcgataaaattaaacgtaacaaagaagccctgctgctgggcctgacctatctggaacgctggtacaatttcagctatggtcaggttaacgtcaaagacctggtgctgtatcatctggatttctttggtaaaggcaacgcaagtccgctggataccctgattgaactgggtaaatccggctttaacaatctgctggcgaaaaacaatgttgacacctacggcatcagtctggcctcccagcatggtaccacggacctgtttagcacgctggaacactatcgtaaagtgttcctgccgaataccagtaacaatgattggtttaaatccgaaacgaaagcgtatattgtggaagaaaaaagcaccatcgaagaagttaaaacgaaacagggtctggcgggcaccaaatacagtattggcgtttatgatcgcatcaccagcgccacgtggaaatatcgcaacatggtgctgccgctgctgaccctgccggaacgctctgtgttcgttattagtacgatgtcctcactgggttttggcgcctacgaccgttatcgctcgagcgatcataaagcgggtaaagccctgaatgattttgtggaagaaaacgctcgtgaaaccgcgaaacgtcagcgcgaccactatgattactggtatcgcattctggatgacaatgcgcgtgaaaaactgtatcgcaacatcctgctgtacgatgcctataaattcggcgatgacaataccgtgggtaaagccacggaagttgcagattttgacaatccgaacccggcgatgcaacatttctttggtccggtcggcaataaagtgggtcataaccagcacggcgcgtatgcgaccggtgatgcagtgtattacatgggctaccgtatgctggataaagacggtgctattacctatacgcatgaaatgacccacgatagtgaccaggatatctacctgggcggttatggtcgtcgctccggtctgggcccggaatttttcgctaaaggtctgctgcaggcgccggatcatccggatgacgcaaccattacgatcaattcaattctgaaacactcgaaaagcgactctaccgaatcgcgtcgcctgcaagttctggatccgaccacgcgcttcaacaatgcggatgacctgaaacagtatgtgcataacatgtttgatgttgtctacatgctggaatatctggaaggcaatagcattctgaaactggacaccaaccagaaacagcaactgctgcgtaaagttacgaatgaatatcacccggacccggatggtaacaaagtgtacgcgaccaatgtggttcgcaacctgacggtcgaagaagtggaacgtctgcgctcattcaacgacctgattgataacaatatcctgtctagtcgtgaatacgcatcgggcaaatatgaacgcaatggttactttaccattaaactgttcgctccgatctacgcagctctgagtaacgacattggtacgccgggtgatctgatgggtcgtcgcatcgcctatgaactgctggcggccaaaggctttaaagatggtatggttccgtatattagcaatcagtacgaagaagaagcgaaacaaaaaggtaaaaccatcaacctgtatggcaaaacccgtggtctggtgacggatgacctggttctggaaaaagtcttcaacaatcaataccatacctggagcgaatttaaaaaagcgatgtatcaggaacgtcaggaccaatttgatcgcctgaataaagttaccttcaacgataccacgcagccgtggcaaacgtttgcgaagaaaaccacgtcctcagtggatgaactgcagaaactgatggacgtcgccgtgcgtaaagatgcagaacataactactaccactggaacaactacaacccggacattgatagcgaagtgcacaaactgaaacgcgcgatcttcaaagcgtacctggaccaaaccaatgacttccgttctagtatcttcgaaaacaaaaaaagatctagatctggatcaagcgggtcatctggagaatcgaagtacggtccgccgtgtccgagttgcccggctccggagtttctgggtggccctagcgtgttcttatttccgccaaagccgaaggacaccctgatgatcagccgcaccccggaggtaacttgcgtcgtcgtggatgtttcccaagaagatccggaggtgcagtttaactggtatgtggacggcgttgaagttcataatgcgaaaaccaagccgcgtgaagagcagttcaacagcacctatcgtgtggtctccgtgttgacggttcttcaccaggattggttgaatggtaaagaatataagtgcaaagtttccaataaaggcctgccgtcgagcattgaaaaaacgattagcaaggcaaagggccaacctcgcgagccgcaagtgtacactctgccgccgagccaagaggaaatgaccaaaaaccaggtttcattgacctgcctggttaagggtttttacccgagcgacatcgccgttgagtgggaatctaacggccagccggagaacaactacaagaccaccccaccggttctggacagcgatggttccttcttcctgtactcccgtctcaccgtggacaaaagccgttggcaagagggaaacgtgttctcttgtagcgtgatgcatgaagcgctgcacaatcattatacgcagaaatctctgagcctttctctgggcaaa

SEQ ID NO: 26 - protein, 1938 aa, synthetic construct
QETAGVHYKYVADSELSSEEKKQLVYDIPTYVENDDETYYLVYKLNSQNQLAELPNTGSKNERQALVAGASLAALGILIFAVSKKKVKNKTVLHLVLVAGIGNGVLVSVHALENHLLLNYNTDYELTSGEKLPLPKEISGYTYIGYIKEGKTTSDFEVSNQEKSAATPTKQQKVDYNVTPNFVDHPSTVQAIQEQTPVSSTKPTEVQVVEKPFSTELINPRKEEKQSSDSQEQLAEHKNLETKKEEKISPKEKTGVNTLNPQDEVLSGQLNKPELLYREETIETKIDFQEEIQENPDLAEGTVRVKQEGKLGKKVEIIRIFSVNKEEVSREIISTSTTAPIPRIVEKGTKKTQIIKEQPETGVEHKDVQSGAIVEPAIQPELSEAVVSDKGVPEVQPALPEAVVSDKGEPEQVATLPEYKGNIEQVKPETPVEKTKEEVPVKPTEETPVNPNEGTTEGTSIQEAENPVQPAEESTTNSEKVSPDTSSENTGEVSSNPSDSTTSVGESNKPEHNDSKNENSEKTVEEVPVNPNEGTVEGTSNQETEKPVQPAEETQTNSGKIANENTGEVSNKPSDSKPPVEESNQPEKNGTATKPENSGNTTSENGQPEPEPSNGNSTEDVSTESNTSNSNGNEEIKQENELDPDKKVEDPEKKLELRNVSDLELYSLSNGTYKQHISLEQVPSNPNSYFVKVKSSSFKDVYLPVASISEERKNDKILYKITAKVEKLQQEIESRYKDNFTFYLAKKGTEETTNFTSFSNLVKAINQNLSGTYRLGASLNANEVELGPDERSYIKDTFTGRLIGEKDGKNYAIYNLKKPLFENLSGATVEKLSLKNVAISGKDDIGSLANEAQNNTKIKQVHVDGVLAGERGIGGLLAKADQSSITESSFKGRIVNTYETKSAYNIGGLVGHLTGDRASINSSKSTVVISSNTNSSDQTVGGISGLVDKDAHIQNSYSEGDINNSQRFGKVAGIAGNLWDRESNSENHAGRLTNVLSDVNVTNGNAISGYHYNGMKITDAFSNKANKVFNVTLEKDEVVSKESFEERGTMLDASQIASKKAEINLLTPPIVEPLSTSGKKDSDFSKIAHYQANRALVYKNIEKLLPFYNKTTIVKYGNLVNENSLLYQKELLSAVMMKDNQVITDIVSNKQTANKLLLHYKDDLSEKLDLKYQNDFAKLAEYSLGNTGLLYTPNQFLYDQTSIIKQVLPDLQKVDYHSEDIRKTLGISPNVKQTELYLEDQFAKTKQQLEDSLKKLLSADAGLASANPVTEGYLVDKIKRNKEALLLGLTYLERWYNFSYGQVNVKDLVLYHLDFFGKGNASPLDTLIELGKSGFNNLLAKNNVDTYGISLASQHGTTDLFSTLEHYRKVFLPNTSNNDWFKSETKAYIVEEKSTIEEVKTKQGLASTKYSIGVYDRITSATWKYRNMVLPLLTLPERSVFVISTMSSLGFGAYDRYRSSDHKAGKALNDFVEENARETAKRQRDHYDYWYRILDDNAREKLYRNILLYDAYKFGDDNTVGKATEVADFDNPNPAMQHFFGPVGNKVGHNQHGAYATGDAVYYMGYRMLDKDGAITYTHEMTHDSDQDIYLGGYGRRSGLGPEFFAKGLLQAPDHPDDATITINSILKHSKSDSTESRRLQVLDPTTRFNNADDLKQYVHNMFDVVYMLEYLEGNSILKLDTNQKQQLLRKVTNEYHPDPDGNKVYATNVVRNLTVEEVERLRSFNDLIDNNILSSREYASGKYERNGYFTIKLFAPIYAALSNDIGTPGDLMGRRIAYELLAAKGFKDGMVPYISNQYEEEAKQKGKTINLYGKTRGLVTDDLVLEKVFNNQYHTWSEFKKAMYQERQDQFDRLNKVTFNDTTQPWQTFAKKTTSSVDELQKLMDVAVRKDAEHNYYHWNNYNPDIDSEVHKLKRAIFKAYLDQTNDFRSSIFENKK

SEQ ID NO: 27 - protein, 1963 aa, synthetic construct
QETAGVHYKYVADSELSSEEKKQLVYDIPTYVENDDETYYLVYKLNSQNQLAELPNTGSKNEMQALVAGASLATLGILIFAVSKKKVKNKTVLHLVLVAGIGNGVLVSVHALENHLLLNYNTDYELTSGEKLPLPKEISGYTYIGYIKEGKTTSDFEVSNQEKSAATPTKQQKVDYNVTPNFVDHPSTVQAIQEQTPVSSTKPTEVQVVEKPFSTELINPRKEEKQSSDSQEQLAEHKNLETKKEEKISPKEKTGVNTLNPQDEVLSGQLNKPELLYREETIETKIDFQEEIQENPDLAEGTVRVKQEGKLGKKVEIVRIFSVNKEEVSREIVSTSTTAPSPRIVEKGTKKTQVIKEQPETGVEHKDVQSGAIVEPAIQPELPEAVVSDKGEPEVQPTLPEAVVTDKGETEVQPESPDTVVSDKGEPEQVATLPEYKGNIEQVKPETPVEKTKEEVPVKPTEEVPVKPTEETPVNPNEGTTEGTSIQEAENPVQPAEESTTNSEKVSPDTSSENTGEVSSNPSDSTTSVGESNKPEHNDSKNENSEKTVEEVPVNPNEGTVEGTSNQETEKPVQPAEETQTNSGKIANENTGEVSNKPSDSKPPVEESNQPEKNGTATKPENSGNTTSENGHPEPEPSNGNSTEDVSTESNTSNSNGNEEIKQENELDPDKKVEDPEKKLELRNVSDLELYSLSNGTYKQHISLEQVPSNPNSYFVKVKSSSFKDVYLPVASISEERKNDKILYKITAKVEKLQQEIESRYKDNFTFYLAKKGTEETTNFTSFSNLVKAINQNLAGTYHLAASLNANEVELANTDNAYIKGTFTGKLIGKNNGKHYAIYNLKKSLFDSLSNATVENLSLKSVNISGKNDIGSLANEAKNGTTINEVHVDGLLGGERGIGGLVAKVDQSNITNSSFTGRIVNTYETKSAYNIGGLVGHLTGDRASINSSKSTVVISSNTNSSDQTVGGIAGLVDKDAHIQNSYSEGDINNSQRFGKVAGIAGNLWDRESNSENHAGRLTNVLSDVNVTNGNAISGYHYNGMKITDAFSNKANKVFNVTLEKDEVVSKESFEERGTMLDASQIASKKAEINLLTPPIVEPLSTSGKKDSDFSKIAHYQANRALVYKNIEKLLPFYNKATIVKYGNLVKENSILYQKELLSAVMMKDDQVITDIISNKQTANKLLLHYKDHSSEKLELKYKDDFANLAEYSIGDSGLLYTPNQFLYDQTSIINQVLPELNRVNYQSDAVRNTLGISPEVKLTELYLEEQFTKTKQDLANSLKKLLSADAGLAGDNPVTRGYLVDKIKNNKEALLLGLTYLERWYNFSYGQVNVKDLVMYHPDFFGKGNTSPLDTLIELGKSGFNNLLAKNNVDTYAISLASHHGTTDLFSTLENYRKVFLPDKTNNDWFKSQTKAYIVEEKSNIEEVKTKQELVGTKYSIGVYDRITSATWKYRNMVLPLLTLPEKSVFVISTISSLGFGAYDRYRNSEHKAGKDLNDFVEENARETAKRQRDHYDYWYRILDNNAREKLYRNILLYDAYKLGDDNTVGKATKVASFDDPNPAMKYFFGPVGNKVGHNGHGAYATGDAVYYMGYRMLDKDGAITYTHEMTHDSDQDIYLGGYGRRSGLGPEFFAKGLLQAPDQPSDATITINSILKHKTSDSTEGQRLQVLDPTTRFNDAADLQNYVHNMFDLIYMLEYLEGQSIVNKLSVYQKMAALRKIENKYVKDPADGNEVYATNVVKELTEAEARNLNSFESLIDHNILSAREYQSGDYERNGYYTIKLFAPIYSALSSEKGTPGDLMGRRMAYELLAAKGFKDGMVPYISNQFEADARANNKTITSYGKTKGLVTDTLVLQKLFNGQYNTWSDFKKAMYKERQDKFNKLNKISFKDPSQPWTRNIIKTIHSVNELQNLMNEAVRKDTETPHWYNYNPEIDSAVHKLKRAIFKAYLDQTNDFRSSIFENKK

SEQ ID NO: 28 - protein, 1793 aa, synthetic construct
QENVAVHYKYVTDTELSGQEKDLIVKDIPKIAEDSESTYYLVYRMDEKAQLGQLPNTGGQNSLTSVLTGGALASIGLLIFVVSKKKGKKKALLNVILVTGMGSGLASSVQAIENQLLLQYNQEYQLSQGDSLPLPRALSGYTYLGYIKQDKEINQQETAARDQKLDYTVQPHFQANEGGQKAGDEQKAPSSTSPADKTIPSQDLSNKKPSGIASVDPQDEVLAGRVNKPELLYKDQEIVTKLDVSEVVQENPDLAEGTIHVKQEGRAGKKIELVRIFTVENQEISREVLSTKVEEALPRIVEKGTKKAVAASEAPQSARKGEPETQAPLPEYTGEQAGAVVAPETAEKPEYTGTQAGAVVEPEQVAPLPEYQGTQAGAIVEPEQVEPEVGGVQSGALVEPETTDKPAYTGEQSGAIVEPEQVPPTPEYTGTQAGAIVDPEIAEKPEYTDTQSGAIVEPETQSSLPEYKGEQAGAIVEPEQVAPLPEYTGNTEQVKPETPTEKPKEKDPEKTLELRNVSDLELYSQTNGTYKQHVSLDGVPSNPDTYFVKVKSSSFKDVYLPVASITAEIKNGQPVYKITAKAEKLQQELENKYVDNFTFYLAKKAREETTTFTSFSNLVKAINQNLSGTYHLAASLNANEVELEPEAKSYIKGTFTGQLIGEKDGKQYAIYNLKKPLFETLSSATVEKLSLKNVSISGKDDIGALSYEAQNGTKIQQVHVDGVLAGERGIGGLLAKAEQSSITESSFKGRIINTYETTAAYNIGGLVGHLTGDKALLTKSKATVAISSNTNSSDQTVAGLAGLVDQDAQIQDSYAEGDINNAKHFGRVAGVAGYLWDRKTNEEQHAGRLTNVLSDVNVTNGNAITGYHYNGMKVKDTFSSKANRVYNVTLVKDEVVSKESFEERGTMLDASQIESKKAAINPLTLPTVEPLSTSGKKDSDFSKVAHYQAKRALAYKNIEKLLPFYNKATIVKYGNLVNENSLLYQKELLSAVMMKDNQVITDIVSNKETANKLLLHYKDHSSEKLNLKYQDDFAKLAEYSLGDTGLLYTPNQFLYDQSSIIKQVLPDLQKIDYHSEAIRKTLGISPKVEQTELYLEDQFAKTKQHLEDSLKKLLSADAGLAGANPVTKGYLVDKIKRNKEALLLGLTYLERWYNFSYGQVNVKDLVLYHLDFFGKGNASPLDTLIELGKSGFNNLLAKNNVDTYGISLANQHGTTDLFSTLENYRKVFLPTTSNNDWFKSETKAYIVEEKSTIEEVKAKQGLAGTKYSVGVYDRITSATWKYRNMVLPLLTLPEKSVFVISTMSSLGFGAYDRYRNSDHKAGKALNDFVEENARETAKRQRDHYDYWYRILDNEGREKLYRTILLYDAYKFGDDTTSGKATLEAKFDSSNPAMKNFFGPVGNKVVHNQHGAYATGDGVYYMSYRMLDKDGAITYTHEMTHDSDQDIYLGGYGRRSGLGPEFFAKGLLQAPDQPSDATITINSILRHSKSDSAEGSRLQVLDPTERFQNASDLQSYVHNMFDLIYMLEYLEGQSIVNKLNVYQKMAALRKIENKYVKDPADGNEVYATNVVKELTEAEAQNLNSFESLIDHNILSAREYQSGEYERNGYYTIKLFAPIFSALSSEKGTPGDLMGRRIAYELLAAKGFKDGMVPYISNQYEEVAKQKGKTINLYGKERGLVTDKLVLDKVFEGKYSSWANFKKAMYKERVDQFENLKQVTFKDPTKPWPSYATKTINSVTELQELMDQAVLQDAVAPRWSNYNPEYDSAVHKLKRAIFKAYLDQTKDFRTSIFKK

SEQ ID NO: 29 - protein, 1793 aa, synthetic construct
QENVAVHYKYVTDTELSRQEKDLIVKDIPKIAEDSESTYYLVYRMDEKAQLGQLPNTGGQHSLTSVLSGGVMASIGLLIFVVSKKKGKKKALLNVILITGMGSGLVSSVQAIENQLLLQYNQEYQLSQGDSLPLPRTLSGYTYLGYIKQDKDASLQETAARGQKPDYTVQPRFQTNEGGQKAGDEQKATSPTTPAEKPIPSQDSSNQNPSGLASVDPQDEVLAGRVNKPELLYKDQEIVTKLDFSEVVQENSELAEGTIRVKQEGHAGKKVEVVRIFTVENQEISREVLSTNVEEALPRIVEKGTKKAVVPSEASQSARKGEPETQASLPEYKGEQAGAIVAPETAEKPEYTGTQAGAVVEPEQVAPQPEYQGTQAGAIVEPEQVEPEVGGVQSGALVEPEMAEKPSYTGEQSGAIVEPEQVPPTQEYTETQAGAVVAPETTETPEYTDNQSGAIVEPEIQSSLPEYKGEQAGAIVEPEQVAPLPEYTGNTEQVKPEAPTEKPKEKDPEKTLELRNVSDLELYSQTNGTYKQHVSLDSVPKNTETYFVKVKSSAVKDVYLPVSSITAETKNGQSVYKITAKAEKLQQELENKYVDNFTFYLAKKATEETTTFTSFSNLVKAIKQNLSGTYYLAASLNANEVELDPDEKSYIKGTFTGQLIGEKDGKQYAIYNLKKPLFETLSGARVEKLSLKNVSISGKDDIGSLAYEAQNGTKIKQVHIDGVLAGERGIGGLLAKADQSSITESSFKGRIINTYETTAAYNIGGLVGHLTGDKALLSKSKATVAISSNTNTSDQTVGGLAGLVDQDAQIQNSYAEGDINNVKHFGRVAGVAGNLWDRTSGDVKYAGSLTNVLSDVNVTNGNAITGYHYNGMKVKDTFSSKANRVYNVTLFKDEVVSRESFEERGTMLDASQIESKKAAINPLTLPTVEPLSTSGKKDSDFSKVTHYQAKRALAYKNIEKLLPFYNKATIVKYGNLVNENSLLYQKELLSAVMMKDNQVITDIVSNKETANKLLLHYKDHSSEKLNLKYQDDFAKLAEYSLGDTGLLYTPNQFLYDQSSIIKQVLPDLQKVDYHSEAIKETLGISPNVKQTELYLEDQFAKTKEQLEDSLKKLLSADAGLAGDNPVTKGYLVDKIKHNKEALLLGLTYLERWYNFSYGQVNVKDLVLYHLDFFGKGNASPLDALIELGKSGFNNLLAKNNVDTYGISLASQHGTTDLFSTLEHYRKVFLPEKSNNDWFKSQTKAYIVEEKSTIEEVKTKQGQTGSKYSIGVYDRITSATWKYRNMVLPLLTLPERSVFVISTMSSLGFGAYDRYRNSEHKAGKALNDFVEENARETAKRQRDHYDYWYRILDNEGREKLYRTILLYDAYKFGDDTTSGKATVEAKFDSSNPAMKNFFGPVGNKVVHNQHGAYATGDGVYYMSYRMLDKDGAITYTHEMTHDSDQDIYLGGYGRRSGLGPEFFAKGLLQAPDQPSDATITINSILKHSTSDSTEGSRLQVLDPTERFQKAADLQNYVHNMFDLIYMLEYLEGQSIVNKLSVYQKMAALRKIENKYVKDPSDGNEVYATNVVKELTAEEAQKLTSFESLIDHNILSAREYQSGEYERNGYYTIKLFAPIFSALSSEKGTPGDLMGRRIAYELLAAKGFKDGMVPYISNQYEEVAKQKGKTINLYGKERGLVTDKLVLDKVFEGKYSSWANFKKAMYKERVDQFENLKQVTFKDPTKPWPSYATKTINSVTELQELMDQAVLQDAVAPRWSDYKPEIDSAVHKLKRAIFKAYLDQTKDFRTSIFKK

SEQ ID NO: 30 - protein, 1952 aa, synthetic construct
QENVSVHYKYVTDTELSSHEKDLIVKDFPNIAEDSESTYYLVYRMDEKAQLGQLPHTGEHNNLVTALTGGALASIGLLIFAVSRKKGNKKALLKVVLITGVGSGLVSSVQAIENQLLLQYNQEYQLSQGDSLPLPRVLSGYTYLGYIKQDKKINQLETVARDQKLDDTVHPHFQSNEGGQNVRDERKNPSPTSPADKSIPSQDSPNQKPSGIASVDPHDEVLAGRLNKPELLYKDQEIVTKLDVLEVVQENPELAEGTIRVKQEGHVGKKVEVVRIFTVENQEITREILSTKVEKSLPRIVEKGTKKAVAPSEAPQSARKGEPETHASLPEYKGEQSGAIVAPEKTDKPSYTGTQSGAIVEPEQVAPQPEYKGIQSGAIVEPEKQEPEVGGAQSGALVEPETADKPSYTGPQSGAVVEPEQVAPQPEYKGTQAGAIVEPETQPSLPEYKGEQSGAIVAPEKTAKPSYTGTQSGAIVEPEKVAPQPEYKGTQAGAIVEPETHASLPEYKGEQSGAIVAPETTEKTEYTGIQSGVIVEPETADKPSYTGTQSGAVVEPEQVAPQPEYTGTQAGTIVEPETLASLPEYKGEQSGAVVAPETADKPEYTGIQSGAIVEPEQAPSKPSYTGTQSGAIVEPEQIAPLPEYTGNIEQAKPENPAEKPKEKDPEKTLELRNVSDLELYSQTNGTYKQHVSLDSVPSNPDTYFVKVKSSSFKDVYLPVASITAEIKNGQSVYKIIAKAEKLQQELENKYVDNFTFYLAKKATEETTTFTSFSNLVKAINKNLSGTYHLAASLNANEVELGPDDRSYIKGTFTGQLMGEKDGKQYAIYNLKKPLFATLRGATVEKLSLKNVSISGKDDIGSLANEATDNTKIKQVHVDGVLAGERGIGGLLAKADQSSITESSFKGRIVNTYETTAAYNIGGLVGHLTGGRASLTKSKATVAISSNTNSSDQTVGGLAGLVDQDAHIQDSYAEGDINNVKHFGRVAGVAGYLWDRKTNEEQHAGRLTNVLSDVNVTNGNAITGYHYNEMKVANTFSNKANRVYNVTLVREEVVSKESFVERGTILDASEVTNKKAEITPLTPPIVEPLSTSGSKESDFSKVKHYQVKRALAYKNIEKLLPFYNKATIVKYGNLVNENSLLYQKELLSAVMMKDDQVITDIVSNKQTANKLLLHYQDHSSETFQIKYQTDFAKLAEYSLGDTGLLYTPNQFLYNQETIIQQVLPELKKVNYHSDAIRNTLGISPKVKQTELYLEEQFAKTKEHLEDSLRKLLSADAGLVENNQVMTGYIVDKIKRNKEALLLGMSYLERWYNFSYGQVNIKDLVLYHLDFFGKGNASPLDTLIELGKSGFNNLLAKNNVDTYGISLASHHGTTDLFSTLENYRKVFLPNTSNNDWFKKQTKAFIVEEKSTIAEVKAKQEQAGTKYSIGVYDRITSSTWKYRNMVLPLLTLPERSVFVISTLSSLGFGAYDRYRNSDYRAGDKLNKFVEENARETAKRQRDHYDYWYRILDNQGREKLYRTILLYDAYKFGDDHTEGKASTIADFENSNPAMQHFFGPVGNKVVHNHHGAYATGDGVYYMSYRMLDKDGAITYTHEMTHDSDQDIYLGGYGRRSGLGPEFFAKGLLQAPDHPNDATITINSILKHSKSDSLEGSRLQVLDPTERFKDASDLQKYVHNMFDLIYLLEYLEGQSIVKKLNVSQKMEALRKIENKYVKDPADGNDVYATNVVKDLTEEEAKKLTSFDSLIDNNILSAREYQVGTYERNGYFTIKLFAPIFSALSSEKGTPGDLMGRRIAYELLAAKGFKDGMVPYISNQYEEIAKQNGQTINLYGKKQGLVTDKLVLEKLFGGQYSSWAAFKKAMYQERVAQFDHLNKVTFKDPTQSWMSNATKTIQRVNELQELMDQAVLKDAEGTRWSDYNPETDSAVHKLKRAVFKAYLDQTNDFRTSIFANKK

SEQ ID NO: 31 - protein, 7 aa, synthetic construct
RSGGGGS